European Patent Application EP 4 763 229 A1, published June 24, 2026. Title: ANTI-GPC3 ANTIBODY DRUG CONJUGATES. Applicant: AbbVie Biotherapeutics Inc. Application EP. The sequence listing filed with the application follows.

SEQUENCE LISTING (117 sequences)

SEQ ID NO: 1 - protein, 120 aa, synthetic construct
EVQLVESGGGLVQPGGSLRLSCAASGFTFSGFGMNWVRQAPGKGLEWVSYTSSSSRTIYYADSVKGRFTISRDNAQNSLYLQMNSLRDEDTAVYYCARDSSGWYDAFDIWGQGTMVTVSS

SEQ ID NO: 2 - protein, 107 aa, synthetic construct
DIQLTQSPSFLSASVGDRVTITCRASQDISSYLAWYQQEPGKAPKLLIYATSTLQSGVPSRFSGSGSGTEFTLTITSLQPEDFATYYCQQLNSYPWTFGQGTKVEIK

SEQ ID NO: 3 - protein, 10 aa, synthetic construct
GFTFSGFGMN

SEQ ID NO: 4 - protein, 17 aa, synthetic construct
YTSSSSRTIYYADSVKG

SEQ ID NO: 5 - protein, 11 aa, synthetic construct
DSSGWYDAFDI

SEQ ID NO: 6 - protein, 11 aa, synthetic construct
RASQDISSYLA

SEQ ID NO: 7 - protein, 7 aa, synthetic construct
ATSTLQS

SEQ ID NO: 8 - protein, 9 aa, synthetic construct
QQLNSYPWT

SEQ ID NO: 9 - protein, 450 aa, synthetic construct
EVQLVESGGGLVQPGGSLRLSCAASGFTFSGFGMNWVRQAPGKGLEWVSYTSSSSRTIYYADSVKGRFTISRDNAQNSLYLQMNSLRDEDTAVYYCARDSSGWYDAFDIWGQGTMVTVSSASTKGPSVFPLAPSSKSTSGGTAALGCLVKDYFPEPVTVSWNSGALTSGVHTFPAVLQSSGLYSLSSVVTVPSSSLGTQTYICNVNHKPSNTKVDKKVEPKSCDKTHTCPPCPAPELLGGPSVFLFPPKPKDTLMISRTPEVTCVVVDVSHEDPEVKFNWYVDGVEVHNAKTKPREEQYNSTYRVVSVLTVLHQDWLNGKEYKCKVSNKALPAPIEKTISKAKGQPREPQVYTLPPSREEMTKNQVSLTCLVKGFYPSDIAVEWESNGQPENNYKTTPPVLDSDGSFFLYSKLTVDKSRWQQGNVFSCSVMHEALHNHYTQKSLSLSPGK

SEQ ID NO: 10 - protein, 214 aa, synthetic construct
DIQLTQSPSFLSASVGDRVTITCRASQDISSYLAWYQQEPGKAPKLLIYATSTLQSGVPSRFSGSGSGTEFTLTITSLQPEDFATYYCQQLNSYPWTFGQGTKVEIKRTVAAPSVFIFPPSDEQLKSGTASVVCLLNNFYPREAKVQWKVDNALQSGNSQESVTEQDSKDSTYSLSSTLTLSKADYEKHKVYACEVTHQGLSSPVTKSFNRGEA

SEQ ID NO: 11 - protein, 449 aa, synthetic construct
EVQLVESGGGLVQPGGSLRLSCAASGFTFSGFGMNWVRQAPGKGLEWVSYTSSSSRTIYYADSVKGRFTISRDNAQNSLYLQMNSLRDEDTAVYYCARDSSGWYDAFDIWGQGTMVTVSSASTKGPSVFPLAPSSKSTSGGTAALGCLVKDYFPEPVTVSWNSGALTSGVHTFPAVLQSSGLYSLSSVVTVPSSSLGTQTYICNVNHKPSNTKVDKKVEPKSCDKTHTCPPCPAPELLGGPSVFLFPPKPKDTLMISRTPEVTCVVVDVSHEDPEVKFNWYVDGVEVHNAKTKPREEQYNSTYRVVSVLTVLHQDWLNGKEYKCKVSNKALPAPIEKTISKAKGQPREPQVYTLPPSREEMTKNQVSLTCLVKGFYPSDIAVEWESNGQPENNYKTTPPVLDSDGSFFLYSKLTVDKSRWQQGNVFSCSVMHEALHNHYTQKSLSLSPG

SEQ ID NO: 12 - protein, 450 aa, synthetic construct
EVQLVESGGGLVQPGGSLRLSCAASGFTFSGFGMNWVRQAPGKGLEWVSYTSSSSRTIYYADSVKGRFTISRDNAQNSLYLQMNSLRDEDTAVYYCARDSSGWYDAFDIWGQGTMVTVSSASTKGPSVFPLAPSSKSTSGGTAALGCLVKDYFPEPVTVSWNSGALTSGVHTFPAVLQSSGLYSLSSVVTVPSSSLGTQTYICNVNHKPSNTKVDKKVEPKSCDKTHTCPPCPAPESTRGPSVFLFPPKPKDTLMISRTPEVTCVVVDVSHEDPEVKFNWYVDGVEVHNAKTKPREEQYNSTYRVVSVLTVLHQDWLNGKEYKCKVSNKALPAPIEKTISKAKGQPREPQVYTLPPSREEMTKNQVSLTCLVKGFYPSDIAVEWESNGQPENNYKTTPPVLDSDGSFFLYSKLTVDKSRWQQGNVFSCSVMHEALHNHYTQKSLSLSPGK

SEQ ID NO: 13 - protein, 449 aa, synthetic construct
EVQLVESGGGLVQPGGSLRLSCAASGFTFSGFGMNWVRQAPGKGLEWVSYTSSSSRTIYYADSVKGRFTISRDNAQNSLYLQMNSLRDEDTAVYYCARDSSGWYDAFDIWGQGTMVTVSSASTKGPSVFPLAPSSKSTSGGTAALGCLVKDYFPEPVTVSWNSGALTSGVHTFPAVLQSSGLYSLSSVVTVPSSSLGTQTYICNVNHKPSNTKVDKKVEPKSCDKTHTCPPCPAPESTRGPSVFLFPPKPKDTLMISRTPEVTCVVVDVSHEDPEVKFNWYVDGVEVHNAKTKPREEQYNSTYRVVSVLTVLHQDWLNGKEYKCKVSNKALPAPIEKTISKAKGQPREPQVYTLPPSREEMTKNQVSLTCLVKGFYPSDIAVEWESNGQPENNYKTTPPVLDSDGSFFLYSKLTVDKSRWQQGNVFSCSVMHEALHNHYTQKSLSLSPG

SEQ ID NO: 14 - protein, 450 aa, synthetic construct
EVQLVESGGGLVQPGGSLRLSCAASGFTFSGFGMNWVRQAPGKGLEWVSYTSSSSRTIYYADSVKGRFTISRDNAQNSLYLQMNSLRDEDTAVYYCARDSSGWYDAFDIWGQGTMVTVSSASTKGPSVFPLAPSSKSTSGGTAALGCLVKDYFPEPVTVSWNSGALTSGVHTFPAVLQSSGLYSLSSVVTVPSSSLGTQTYICNVNHKPSNTKVDKKVEPKSCDKTHTCPPCPAPEAAGGPSVFLFPPKPKDTLMISRTPEVTCVVVDVSHEDPEVKFNWYVDGVEVHNAKTKPREEQYNSTYRVVSVLTVLHQDWLNGKEYKCKVSNKALPAPIEKTISKAKGQPREPQVYTLPPSREEMTKNQVSLTCLVKGFYPSDIAVEWESNGQPENNYKTTPPVLDSDGSFFLYSKLTVDKSRWQQGNVFSCSVMHEALHNHYTQKSLSLSPGK

SEQ ID NO: 15 - protein, 449 aa, synthetic construct
EVQLVESGGGLVQPGGSLRLSCAASGFTFSGFGMNWVRQAPGKGLEWVSYTSSSSRTIYYADSVKGRFTISRDNAQNSLYLQMNSLRDEDTAVYYCARDSSGWYDAFDIWGQGTMVTVSSASTKGPSVFPLAPSSKSTSGGTAALGCLVKDYFPEPVTVSWNSGALTSGVHTFPAVLQSSGLYSLSSVVTVPSSSLGTQTYICNVNHKPSNTKVDKKVEPKSCDKTHTCPPCPAPEAAGGPSVFLFPPKPKDTLMISRTPEVTCVVVDVSHEDPEVKFNWYVDGVEVHNAKTKPREEQYNSTYRVVSVLTVLHQDWLNGKEYKCKVSNKALPAPIEKTISKAKGQPREPQVYTLPPSREEMTKNQVSLTCLVKGFYPSDIAVEWESNGQPENNYKTTPPVLDSDGSFFLYSKLTVDKSRWQQGNVFSCSVMHEALHNHYTQKSLSLSPG

SEQ ID NO: 16 - protein, 450 aa, synthetic construct
EVQLVESGGGLVQPGGSLRLSCAASGFTFSGFGMNWVRQAPGKGLEWVSYTSSSSRTIYYADSVKGRFTISRDNAQNSLYLQMNSLRDEDTAVYYCARDSSGWYDAFDIWGQGTMVTVSSASTKGPSVFPLAPSSKSTSGGTAALGCLVKDYFPEPVTVSWNSGALTSGVHTFPAVLQSSGLYSLSSVVTVPSSSLGTQTYICNVNHKPSNTKVDKKVEPKSCDKTHTCPPCPAPELLGGPSVFLFPPKPKDTLYITREPEVTCVVVDVSHEDPEVKFNWYVDGVEVHNAKTKPREEQYNSTYRVVSVLTVLHQDWLNGKEYKCKVSNKALPAPIEKTISKAKGQPREPQVYTLPPSREEMTKNQVSLTCLVKGFYPSDIAVEWESNGQPENNYKTTPPVLDSDGSFFLYSKLTVDKSRWQQGNVFSCSVMHEALHNHYTQKSLSLSPGK

SEQ ID NO: 17 - protein, 449 aa, synthetic construct
EVQLVESGGGLVQPGGSLRLSCAASGFTFSGFGMNWVRQAPGKGLEWVSYTSSSSRTIYYADSVKGRFTISRDNAQNSLYLQMNSLRDEDTAVYYCARDSSGWYDAFDIWGQGTMVTVSSASTKGPSVFPLAPSSKSTSGGTAALGCLVKDYFPEPVTVSWNSGALTSGVHTFPAVLQSSGLYSLSSVVTVPSSSLGTQTYICNVNHKPSNTKVDKKVEPKSCDKTHTCPPCPAPELLGGPSVFLFPPKPKDTLYITREPEVTCVVVDVSHEDPEVKFNWYVDGVEVHNAKTKPREEQYNSTYRVVSVLTVLHQDWLNGKEYKCKVSNKALPAPIEKTISKAKGQPREPQVYTLPPSREEMTKNQVSLTCLVKGFYPSDIAVEWESNGQPENNYKTTPPVLDSDGSFFLYSKLTVDKSRWQQGNVFSCSVMHEALHNHYTQKSLSLSPG

SEQ ID NO: 18 - protein, 450 aa, synthetic construct
EVQLVESGGGLVQPGGSLRLSCAASGFTFSGFGMNWVRQAPGKGLEWVSYTSSSSRTIYYADSVKGRFTISRDNAQNSLYLQMNSLRDEDTAVYYCARDSSGWYDAFDIWGQGTMVTVSSASTKGPSVFPLAPSSKSTSGGTAALGCLVKDYFPEPVTVSWNSGALTSGVHTFPAVLQSSGLYSLSSVVTVPSSSLGTQTYICNVNHKPSNTKVDKKVEPKSCDKTHTCPPCPAPESTRGPSVFLFPPKPKDTLYITREPEVTCVVVDVSHEDPEVKFNWYVDGVEVHNAKTKPREEQYNSTYRVVSVLTVLHQDWLNGKEYKCKVSNKALPAPIEKTISKAKGQPREPQVYTLPPSREEMTKNQVSLTCLVKGFYPSDIAVEWESNGQPENNYKTTPPVLDSDGSFFLYSKLTVDKSRWQQGNVFSCSVMHEALHNHYTQKSLSLSPGK

SEQ ID NO: 19 - protein, 449 aa, synthetic construct
EVQLVESGGGLVQPGGSLRLSCAASGFTFSGFGMNWVRQAPGKGLEWVSYTSSSSRTIYYADSVKGRFTISRDNAQNSLYLQMNSLRDEDTAVYYCARDSSGWYDAFDIWGQGTMVTVSSASTKGPSVFPLAPSSKSTSGGTAALGCLVKDYFPEPVTVSWNSGALTSGVHTFPAVLQSSGLYSLSSVVTVPSSSLGTQTYICNVNHKPSNTKVDKKVEPKSCDKTHTCPPCPAPESTRGPSVFLFPPKPKDTLYITREPEVTCVVVDVSHEDPEVKFNWYVDGVEVHNAKTKPREEQYNSTYRVVSVLTVLHQDWLNGKEYKCKVSNKALPAPIEKTISKAKGQPREPQVYTLPPSREEMTKNQVSLTCLVKGFYPSDIAVEWESNGQPENNYKTTPPVLDSDGSFFLYSKLTVDKSRWQQGNVFSCSVMHEALHNHYTQKSLSLSPG

SEQ ID NO: 20 - protein, 450 aa, synthetic construct
EVQLVESGGGLVQPGGSLRLSCAASGFTFSGFGMNWVRQAPGKGLEWVSYTSSSSRTIYYADSVKGRFTISRDNAQNSLYLQMNSLRDEDTAVYYCARDSSGWYDAFDIWGQGTMVTVSSASTKGPSVFPLAPSSKSTSGGTAALGCLVKDYFPEPVTVSWNSGALTSGVHTFPAVLQSSGLYSLSSVVTVPSSSLGTQTYICNVNHKPSNTKVDKKVEPKSCDKTHTCPPCPAPEAAGGPSVFLFPPKPKDTLYITREPEVTCVVVDVSHEDPEVKFNWYVDGVEVHNAKTKPREEQYNSTYRVVSVLTVLHQDWLNGKEYKCKVSNKALPAPIEKTISKAKGQPREPQVYTLPPSREEMTKNQVSLTCLVKGFYPSDIAVEWESNGQPENNYKTTPPVLDSDGSFFLYSKLTVDKSRWQQGNVFSCSVMHEALHNHYTQKSLSLSPGK

SEQ ID NO: 21 - protein, 449 aa, synthetic construct
EVQLVESGGGLVQPGGSLRLSCAASGFTFSGFGMNWVRQAPGKGLEWVSYTSSSSRTIYYADSVKGRFTISRDNAQNSLYLQMNSLRDEDTAVYYCARDSSGWYDAFDIWGQGTMVTVSSASTKGPSVFPLAPSSKSTSGGTAALGCLVKDYFPEPVTVSWNSGALTSGVHTFPAVLQSSGLYSLSSVVTVPSSSLGTQTYICNVNHKPSNTKVDKKVEPKSCDKTHTCPPCPAPEAAGGPSVFLFPPKPKDTLYITREPEVTCVVVDVSHEDPEVKFNWYVDGVEVHNAKTKPREEQYNSTYRVVSVLTVLHQDWLNGKEYKCKVSNKALPAPIEKTISKAKGQPREPQVYTLPPSREEMTKNQVSLTCLVKGFYPSDIAVEWESNGQPENNYKTTPPVLDSDGSFFLYSKLTVDKSRWQQGNVFSCSVMHEALHNHYTQKSLSLSPG

SEQ ID NO: 22 - protein, 450 aa, synthetic construct
EVQLVESGGGLVQPGGSLRLSCAASGFTFSGFGMNWVRQAPGKGLEWVSYTSSSSRTIYYADSVKGRFTISRDNAQNSLYLQMNSLRDEDTAVYYCARDSSGWYDAFDIWGQGTMVTVSSASTKGPSVFPLAPSSKSTSGGTAALGCLVKDYFPEPVTVSWNSGALTSGVHTFPAVLQSSGLYSLSSVVTVPSSSLGTQTYICNVNHKPSNTKVDKKVEPKSCDKTHTCPPCPAPELLGGPSVFLFPPKPKDTLMISRTPEVTCVVVDVSHEDPEVKFNWYVDGVEVHNAKTKPREEQYNSTYRVVSVLTVLHRDWLNGKEYKCKVSNKALPAPIEKTISKAKGQPREPQVYTLPPSREEMTKNQVSLTCLVKGFYPSDIAVEWESNGQPENNYKTTPPVLDSDGSFFLYSKLTVDKSRWQQGNVFSCSVEHEALHWHYTQKSLSLSPGK

SEQ ID NO: 23 - protein, 449 aa, synthetic construct
EVQLVESGGGLVQPGGSLRLSCAASGFTFSGFGMNWVRQAPGKGLEWVSYTSSSSRTIYYADSVKGRFTISRDNAQNSLYLQMNSLRDEDTAVYYCARDSSGWYDAFDIWGQGTMVTVSSASTKGPSVFPLAPSSKSTSGGTAALGCLVKDYFPEPVTVSWNSGALTSGVHTFPAVLQSSGLYSLSSVVTVPSSSLGTQTYICNVNHKPSNTKVDKKVEPKSCDKTHTCPPCPAPELLGGPSVFLFPPKPKDTLMISRTPEVTCVVVDVSHEDPEVKFNWYVDGVEVHNAKTKPREEQYNSTYRVVSVLTVLHRDWLNGKEYKCKVSNKALPAPIEKTISKAKGQPREPQVYTLPPSREEMTKNQVSLTCLVKGFYPSDIAVEWESNGQPENNYKTTPPVLDSDGSFFLYSKLTVDKSRWQQGNVFSCSVEHEALHWHYTQKSLSLSPG

SEQ ID NO: 24 - protein, 450 aa, synthetic construct
EVQLVESGGGLVQPGGSLRLSCAASGFTFSGFGMNWVRQAPGKGLEWVSYTSSSSRTIYYADSVKGRFTISRDNAQNSLYLQMNSLRDEDTAVYYCARDSSGWYDAFDIWGQGTMVTVSSASTKGPSVFPLAPSSKSTSGGTAALGCLVKDYFPEPVTVSWNSGALTSGVHTFPAVLQSSGLYSLSSVVTVPSSSLGTQTYICNVNHKPSNTKVDKKVEPKSCDKTHTCPPCPAPESTRGPSVFLFPPKPKDTLMISRTPEVTCVVVDVSHEDPEVKFNWYVDGVEVHNAKTKPREEQYNSTYRVVSVLTVLHRDWLNGKEYKCKVSNKALPAPIEKTISKAKGQPREPQVYTLPPSREEMTKNQVSLTCLVKGFYPSDIAVEWESNGQPENNYKTTPPVLDSDGSFFLYSKLTVDKSRWQQGNVFSCSVEHEALHWHYTQKSLSLSPGK

SEQ ID NO: 25 - protein, 449 aa, synthetic construct
EVQLVESGGGLVQPGGSLRLSCAASGFTFSGFGMNWVRQAPGKGLEWVSYTSSSSRTIYYADSVKGRFTISRDNAQNSLYLQMNSLRDEDTAVYYCARDSSGWYDAFDIWGQGTMVTVSSASTKGPSVFPLAPSSKSTSGGTAALGCLVKDYFPEPVTVSWNSGALTSGVHTFPAVLQSSGLYSLSSVVTVPSSSLGTQTYICNVNHKPSNTKVDKKVEPKSCDKTHTCPPCPAPESTRGPSVFLFPPKPKDTLMISRTPEVTCVVVDVSHEDPEVKFNWYVDGVEVHNAKTKPREEQYNSTYRVVSVLTVLHRDWLNGKEYKCKVSNKALPAPIEKTISKAKGQPREPQVYTLPPSREEMTKNQVSLTCLVKGFYPSDIAVEWESNGQPENNYKTTPPVLDSDGSFFLYSKLTVDKSRWQQGNVFSCSVEHEALHWHYTQKSLSLSPG

SEQ ID NO: 26 - protein, 450 aa, synthetic construct
EVQLVESGGGLVQPGGSLRLSCAASGFTFSGFGMNWVRQAPGKGLEWVSYTSSSSRTIYYADSVKGRFTISRDNAQNSLYLQMNSLRDEDTAVYYCARDSSGWYDAFDIWGQGTMVTVSSASTKGPSVFPLAPSSKSTSGGTAALGCLVKDYFPEPVTVSWNSGALTSGVHTFPAVLQSSGLYSLSSVVTVPSSSLGTQTYICNVNHKPSNTKVDKKVEPKSCDKTHTCPPCPAPEAAGGPSVFLFPPKPKDTLMISRTPEVTCVVVDVSHEDPEVKFNWYVDGVEVHNAKTKPREEQYNSTYRVVSVLTVLHRDWLNGKEYKCKVSNKALPAPIEKTISKAKGQPREPQVYTLPPSREEMTKNQVSLTCLVKGFYPSDIAVEWESNGQPENNYKTTPPVLDSDGSFFLYSKLTVDKSRWQQGNVFSCSVEHEALHWHYTQKSLSLSPGK

SEQ ID NO: 27 - protein, 449 aa, synthetic construct
EVQLVESGGGLVQPGGSLRLSCAASGFTFSGFGMNWVRQAPGKGLEWVSYTSSSSRTIYYADSVKGRFTISRDNAQNSLYLQMNSLRDEDTAVYYCARDSSGWYDAFDIWGQGTMVTVSSASTKGPSVFPLAPSSKSTSGGTAALGCLVKDYFPEPVTVSWNSGALTSGVHTFPAVLQSSGLYSLSSVVTVPSSSLGTQTYICNVNHKPSNTKVDKKVEPKSCDKTHTCPPCPAPEAAGGPSVFLFPPKPKDTLMISRTPEVTCVVVDVSHEDPEVKFNWYVDGVEVHNAKTKPREEQYNSTYRVVSVLTVLHRDWLNGKEYKCKVSNKALPAPIEKTISKAKGQPREPQVYTLPPSREEMTKNQVSLTCLVKGFYPSDIAVEWESNGQPENNYKTTPPVLDSDGSFFLYSKLTVDKSRWQQGNVFSCSVEHEALHWHYTQKSLSLSPG

SEQ ID NO: 28 - protein, 450 aa, synthetic construct
EVQLVESGGGLVQPGGSLRLSCAASGFTFSGFGMNWVRQAPGKGLEWVSYTSSSSRTIYYADSVKGRFTISRDNAQNSLYLQMNSLRDEDTAVYYCARDSSGWYDAFDIWGQGTMVTVSSASTKGPSVFPLAPSSKSTSGGTAALGCLVKDYFPEPVTVSWNSGALTSGVHTFPAVLQSSGLYSLSSVVTVPSSSLGTQTYICNVNHKPSNTKVDKKVEPKSCDKTHTCPPCPAPELLGGPSVFLFPPKPKDTLMISRTPEVTCVVVDVSHEDPEVKFNWYVDGVEVHNAKTKPREEQYNSTYRVVSVLTVLHQDWLNGKEYKCKVSNKALPAPIEKTISKAKGQPREPQVYTLPPSREEMTKNQVSLTCLVKGFYPSDIAVEWESNGQPENNYKTTPPVLDSDGSFFLYSKLTVDKSRWQQGNVFSCSVLHEALHSHYTQKSLSLSPGK

SEQ ID NO: 29 - protein, 449 aa, synthetic construct
EVQLVESGGGLVQPGGSLRLSCAASGFTFSGFGMNWVRQAPGKGLEWVSYTSSSSRTIYYADSVKGRFTISRDNAQNSLYLQMNSLRDEDTAVYYCARDSSGWYDAFDIWGQGTMVTVSSASTKGPSVFPLAPSSKSTSGGTAALGCLVKDYFPEPVTVSWNSGALTSGVHTFPAVLQSSGLYSLSSVVTVPSSSLGTQTYICNVNHKPSNTKVDKKVEPKSCDKTHTCPPCPAPELLGGPSVFLFPPKPKDTLMISRTPEVTCVVVDVSHEDPEVKFNWYVDGVEVHNAKTKPREEQYNSTYRVVSVLTVLHQDWLNGKEYKCKVSNKALPAPIEKTISKAKGQPREPQVYTLPPSREEMTKNQVSLTCLVKGFYPSDIAVEWESNGQPENNYKTTPPVLDSDGSFFLYSKLTVDKSRWQQGNVFSCSVLHEALHSHYTQKSLSLSPG

SEQ ID NO: 30 - protein, 450 aa, synthetic construct
EVQLVESGGGLVQPGGSLRLSCAASGFTFSGFGMNWVRQAPGKGLEWVSYTSSSSRTIYYADSVKGRFTISRDNAQNSLYLQMNSLRDEDTAVYYCARDSSGWYDAFDIWGQGTMVTVSSASTKGPSVFPLAPSSKSTSGGTAALGCLVKDYFPEPVTVSWNSGALTSGVHTFPAVLQSSGLYSLSSVVTVPSSSLGTQTYICNVNHKPSNTKVDKKVEPKSCDKTHTCPPCPAPESTRGPSVFLFPPKPKDTLMISRTPEVTCVVVDVSHEDPEVKFNWYVDGVEVHNAKTKPREEQYNSTYRVVSVLTVLHQDWLNGKEYKCKVSNKALPAPIEKTISKAKGQPREPQVYTLPPSREEMTKNQVSLTCLVKGFYPSDIAVEWESNGQPENNYKTTPPVLDSDGSFFLYSKLTVDKSRWQQGNVFSCSVLHEALHSHYTQKSLSLSPGK

SEQ ID NO: 31 - protein, 449 aa, synthetic construct
EVQLVESGGGLVQPGGSLRLSCAASGFTFSGFGMNWVRQAPGKGLEWVSYTSSSSRTIYYADSVKGRFTISRDNAQNSLYLQMNSLRDEDTAVYYCARDSSGWYDAFDIWGQGTMVTVSSASTKGPSVFPLAPSSKSTSGGTAALGCLVKDYFPEPVTVSWNSGALTSGVHTFPAVLQSSGLYSLSSVVTVPSSSLGTQTYICNVNHKPSNTKVDKKVEPKSCDKTHTCPPCPAPESTRGPSVFLFPPKPKDTLMISRTPEVTCVVVDVSHEDPEVKFNWYVDGVEVHNAKTKPREEQYNSTYRVVSVLTVLHQDWLNGKEYKCKVSNKALPAPIEKTISKAKGQPREPQVYTLPPSREEMTKNQVSLTCLVKGFYPSDIAVEWESNGQPENNYKTTPPVLDSDGSFFLYSKLTVDKSRWQQGNVFSCSVLHEALHSHYTQKSLSLSPG

SEQ ID NO: 32 - protein, 450 aa, synthetic construct
EVQLVESGGGLVQPGGSLRLSCAASGFTFSGFGMNWVRQAPGKGLEWVSYTSSSSRTIYYADSVKGRFTISRDNAQNSLYLQMNSLRDEDTAVYYCARDSSGWYDAFDIWGQGTMVTVSSASTKGPSVFPLAPSSKSTSGGTAALGCLVKDYFPEPVTVSWNSGALTSGVHTFPAVLQSSGLYSLSSVVTVPSSSLGTQTYICNVNHKPSNTKVDKKVEPKSCDKTHTCPPCPAPEAAGGPSVFLFPPKPKDTLMISRTPEVTCVVVDVSHEDPEVKFNWYVDGVEVHNAKTKPREEQYNSTYRVVSVLTVLHQDWLNGKEYKCKVSNKALPAPIEKTISKAKGQPREPQVYTLPPSREEMTKNQVSLTCLVKGFYPSDIAVEWESNGQPENNYKTTPPVLDSDGSFFLYSKLTVDKSRWQQGNVFSCSVLHEALHSHYTQKSLSLSPGK

SEQ ID NO: 33 - protein, 449 aa, synthetic construct
EVQLVESGGGLVQPGGSLRLSCAASGFTFSGFGMNWVRQAPGKGLEWVSYTSSSSRTIYYADSVKGRFTISRDNAQNSLYLQMNSLRDEDTAVYYCARDSSGWYDAFDIWGQGTMVTVSSASTKGPSVFPLAPSSKSTSGGTAALGCLVKDYFPEPVTVSWNSGALTSGVHTFPAVLQSSGLYSLSSVVTVPSSSLGTQTYICNVNHKPSNTKVDKKVEPKSCDKTHTCPPCPAPEAAGGPSVFLFPPKPKDTLMISRTPEVTCVVVDVSHEDPEVKFNWYVDGVEVHNAKTKPREEQYNSTYRVVSVLTVLHQDWLNGKEYKCKVSNKALPAPIEKTISKAKGQPREPQVYTLPPSREEMTKNQVSLTCLVKGFYPSDIAVEWESNGQPENNYKTTPPVLDSDGSFFLYSKLTVDKSRWQQGNVFSCSVLHEALHSHYTQKSLSLSPG

SEQ ID NO: 34 - protein, 450 aa, synthetic construct
EVQLVESGGGLVQPGGSLRLSCAASGFTFSGFGMNWVRQAPGKGLEWVSYTSSSSRTIYYADSVKGRFTISRDNAQNSLYLQMNSLRDEDTAVYYCARDSSGWYDAFDIWGQGTMVTVSSASTKGPSVFPLAPSSKSTSGGTAALGCLVKDYFPEPVTVSWNSGALTSGVHTFPAVLQSSGLYSLSSVVTVPSSSLGTQTYICNVNHKPSNTKVDKKVEPKSCDKTHTCPPCPAPELLGGPSVFLFPPKPKDQLMISRTPEVTCVVVDVSHEDPEVKFNWYVDGVEVHNAKTKPREEQYNSTYRVVSVLTVLHQDWLNGKEYKCKVSNKALPAPIEKTISKAKGQPREPQVYTLPPSREEMTKNQVSLTCLVKGFYPSDIAVEWESNGQPENNYKTTPPVLDSDGSFFLYSKLTVDKSRWQQGNVFSCSVLHEALHNHYTQKSLSLSPGK

SEQ ID NO: 35 - protein, 449 aa, synthetic construct
EVQLVESGGGLVQPGGSLRLSCAASGFTFSGFGMNWVRQAPGKGLEWVSYTSSSSRTIYYADSVKGRFTISRDNAQNSLYLQMNSLRDEDTAVYYCARDSSGWYDAFDIWGQGTMVTVSSASTKGPSVFPLAPSSKSTSGGTAALGCLVKDYFPEPVTVSWNSGALTSGVHTFPAVLQSSGLYSLSSVVTVPSSSLGTQTYICNVNHKPSNTKVDKKVEPKSCDKTHTCPPCPAPELLGGPSVFLFPPKPKDQLMISRTPEVTCVVVDVSHEDPEVKFNWYVDGVEVHNAKTKPREEQYNSTYRVVSVLTVLHQDWLNGKEYKCKVSNKALPAPIEKTISKAKGQPREPQVYTLPPSREEMTKNQVSLTCLVKGFYPSDIAVEWESNGQPENNYKTTPPVLDSDGSFFLYSKLTVDKSRWQQGNVFSCSVLHEALHNHYTQKSLSLSPG

SEQ ID NO: 36 - protein, 450 aa, synthetic construct
EVQLVESGGGLVQPGGSLRLSCAASGFTFSGFGMNWVRQAPGKGLEWVSYTSSSSRTIYYADSVKGRFTISRDNAQNSLYLQMNSLRDEDTAVYYCARDSSGWYDAFDIWGQGTMVTVSSASTKGPSVFPLAPSSKSTSGGTAALGCLVKDYFPEPVTVSWNSGALTSGVHTFPAVLQSSGLYSLSSVVTVPSSSLGTQTYICNVNHKPSNTKVDKKVEPKSCDKTHTCPPCPAPESTRGPSVFLFPPKPKDQLMISRTPEVTCVVVDVSHEDPEVKFNWYVDGVEVHNAKTKPREEQYNSTYRVVSVLTVLHQDWLNGKEYKCKVSNKALPAPIEKTISKAKGQPREPQVYTLPPSREEMTKNQVSLTCLVKGFYPSDIAVEWESNGQPENNYKTTPPVLDSDGSFFLYSKLTVDKSRWQQGNVFSCSVLHEALHNHYTQKSLSLSPGK

SEQ ID NO: 37 - protein, 449 aa, synthetic construct
EVQLVESGGGLVQPGGSLRLSCAASGFTFSGFGMNWVRQAPGKGLEWVSYTSSSSRTIYYADSVKGRFTISRDNAQNSLYLQMNSLRDEDTAVYYCARDSSGWYDAFDIWGQGTMVTVSSASTKGPSVFPLAPSSKSTSGGTAALGCLVKDYFPEPVTVSWNSGALTSGVHTFPAVLQSSGLYSLSSVVTVPSSSLGTQTYICNVNHKPSNTKVDKKVEPKSCDKTHTCPPCPAPESTRGPSVFLFPPKPKDQLMISRTPEVTCVVVDVSHEDPEVKFNWYVDGVEVHNAKTKPREEQYNSTYRVVSVLTVLHQDWLNGKEYKCKVSNKALPAPIEKTISKAKGQPREPQVYTLPPSREEMTKNQVSLTCLVKGFYPSDIAVEWESNGQPENNYKTTPPVLDSDGSFFLYSKLTVDKSRWQQGNVFSCSVLHEALHNHYTQKSLSLSPG

SEQ ID NO: 38 - protein, 450 aa, synthetic construct
EVQLVESGGGLVQPGGSLRLSCAASGFTFSGFGMNWVRQAPGKGLEWVSYTSSSSRTIYYADSVKGRFTISRDNAQNSLYLQMNSLRDEDTAVYYCARDSSGWYDAFDIWGQGTMVTVSSASTKGPSVFPLAPSSKSTSGGTAALGCLVKDYFPEPVTVSWNSGALTSGVHTFPAVLQSSGLYSLSSVVTVPSSSLGTQTYICNVNHKPSNTKVDKKVEPKSCDKTHTCPPCPAPEAAGGPSVFLFPPKPKDQLMISRTPEVTCVVVDVSHEDPEVKFNWYVDGVEVHNAKTKPREEQYNSTYRVVSVLTVLHQDWLNGKEYKCKVSNKALPAPIEKTISKAKGQPREPQVYTLPPSREEMTKNQVSLTCLVKGFYPSDIAVEWESNGQPENNYKTTPPVLDSDGSFFLYSKLTVDKSRWQQGNVFSCSVLHEALHNHYTQKSLSLSPGK

SEQ ID NO: 39 - protein, 449 aa, synthetic construct
EVQLVESGGGLVQPGGSLRLSCAASGFTFSGFGMNWVRQAPGKGLEWVSYTSSSSRTIYYADSVKGRFTISRDNAQNSLYLQMNSLRDEDTAVYYCARDSSGWYDAFDIWGQGTMVTVSSASTKGPSVFPLAPSSKSTSGGTAALGCLVKDYFPEPVTVSWNSGALTSGVHTFPAVLQSSGLYSLSSVVTVPSSSLGTQTYICNVNHKPSNTKVDKKVEPKSCDKTHTCPPCPAPEAAGGPSVFLFPPKPKDQLMISRTPEVTCVVVDVSHEDPEVKFNWYVDGVEVHNAKTKPREEQYNSTYRVVSVLTVLHQDWLNGKEYKCKVSNKALPAPIEKTISKAKGQPREPQVYTLPPSREEMTKNQVSLTCLVKGFYPSDIAVEWESNGQPENNYKTTPPVLDSDGSFFLYSKLTVDKSRWQQGNVFSCSVLHEALHNHYTQKSLSLSPG

SEQ ID NO: 40 - protein, 450 aa, synthetic construct
EVQLVESGGGLVQPGGSLRLSCAASGFTFSGFGMNWVRQAPGKGLEWVSYTSSSSRTIYYADSVKGRFTISRDNAQNSLYLQMNSLRDEDTAVYYCARDSSGWYDAFDIWGQGTMVTVSSASTKGPSVFPLAPSSKSTSGGTAALGCLVKDYFPEPVTVSWNSGALTSGVHTFPAVLQSSGLYSLSSVVTVPSSSLGTQTYICNVNHKPSNTKVDKKVEPKSCDKTHTCPPCPAPELLGGPSVFLFPPKPKDTLMISRTPEVTCVVVDVSHEDPEVKFNWYVDGVEVHNAKTKPREEQYNSTYRVVSVLTVDHHDWLNGKEYKCKVSNKALPAPIEKTISKAKGQPREPQVYTLPPSREEMTKNQVSLTCLVKGFYPSDIAVEWESNGQPENNYKTTPPVLDSDGSFFLYSKLTVDKSRWQQGNVFSCSVMHEALHSHYTQKSLSLSPGK

SEQ ID NO: 41 - protein, 449 aa, synthetic construct
EVQLVESGGGLVQPGGSLRLSCAASGFTFSGFGMNWVRQAPGKGLEWVSYTSSSSRTIYYADSVKGRFTISRDNAQNSLYLQMNSLRDEDTAVYYCARDSSGWYDAFDIWGQGTMVTVSSASTKGPSVFPLAPSSKSTSGGTAALGCLVKDYFPEPVTVSWNSGALTSGVHTFPAVLQSSGLYSLSSVVTVPSSSLGTQTYICNVNHKPSNTKVDKKVEPKSCDKTHTCPPCPAPELLGGPSVFLFPPKPKDTLMISRTPEVTCVVVDVSHEDPEVKFNWYVDGVEVHNAKTKPREEQYNSTYRVVSVLTVDHHDWLNGKEYKCKVSNKALPAPIEKTISKAKGQPREPQVYTLPPSREEMTKNQVSLTCLVKGFYPSDIAVEWESNGQPENNYKTTPPVLDSDGSFFLYSKLTVDKSRWQQGNVFSCSVMHEALHSHYTQKSLSLSPG

SEQ ID NO: 42 - protein, 450 aa, synthetic construct
EVQLVESGGGLVQPGGSLRLSCAASGFTFSGFGMNWVRQAPGKGLEWVSYTSSSSRTIYYADSVKGRFTISRDNAQNSLYLQMNSLRDEDTAVYYCARDSSGWYDAFDIWGQGTMVTVSSASTKGPSVFPLAPSSKSTSGGTAALGCLVKDYFPEPVTVSWNSGALTSGVHTFPAVLQSSGLYSLSSVVTVPSSSLGTQTYICNVNHKPSNTKVDKKVEPKSCDKTHTCPPCPAPESTRGPSVFLFPPKPKDTLMISRTPEVTCVVVDVSHEDPEVKFNWYVDGVEVHNAKTKPREEQYNSTYRVVSVLTVDHHDWLNGKEYKCKVSNKALPAPIEKTISKAKGQPREPQVYTLPPSREEMTKNQVSLTCLVKGFYPSDIAVEWESNGQPENNYKTTPPVLDSDGSFFLYSKLTVDKSRWQQGNVFSCSVMHEALHSHYTQKSLSLSPGK

SEQ ID NO: 43 - protein, 449 aa, synthetic construct
EVQLVESGGGLVQPGGSLRLSCAASGFTFSGFGMNWVRQAPGKGLEWVSYTSSSSRTIYYADSVKGRFTISRDNAQNSLYLQMNSLRDEDTAVYYCARDSSGWYDAFDIWGQGTMVTVSSASTKGPSVFPLAPSSKSTSGGTAALGCLVKDYFPEPVTVSWNSGALTSGVHTFPAVLQSSGLYSLSSVVTVPSSSLGTQTYICNVNHKPSNTKVDKKVEPKSCDKTHTCPPCPAPESTRGPSVFLFPPKPKDTLMISRTPEVTCVVVDVSHEDPEVKFNWYVDGVEVHNAKTKPREEQYNSTYRVVSVLTVDHHDWLNGKEYKCKVSNKALPAPIEKTISKAKGQPREPQVYTLPPSREEMTKNQVSLTCLVKGFYPSDIAVEWESNGQPENNYKTTPPVLDSDGSFFLYSKLTVDKSRWQQGNVFSCSVMHEALHSHYTQKSLSLSPG

SEQ ID NO: 44 - protein, 450 aa, synthetic construct
EVQLVESGGGLVQPGGSLRLSCAASGFTFSGFGMNWVRQAPGKGLEWVSYTSSSSRTIYYADSVKGRFTISRDNAQNSLYLQMNSLRDEDTAVYYCARDSSGWYDAFDIWGQGTMVTVSSASTKGPSVFPLAPSSKSTSGGTAALGCLVKDYFPEPVTVSWNSGALTSGVHTFPAVLQSSGLYSLSSVVTVPSSSLGTQTYICNVNHKPSNTKVDKKVEPKSCDKTHTCPPCPAPEAAGGPSVFLFPPKPKDTLMISRTPEVTCVVVDVSHEDPEVKFNWYVDGVEVHNAKTKPREEQYNSTYRVVSVLTVDHHDWLNGKEYKCKVSNKALPAPIEKTISKAKGQPREPQVYTLPPSREEMTKNQVSLTCLVKGFYPSDIAVEWESNGQPENNYKTTPPVLDSDGSFFLYSKLTVDKSRWQQGNVFSCSVMHEALHSHYTQKSLSLSPGK

SEQ ID NO: 45 - protein, 449 aa, synthetic construct
EVQLVESGGGLVQPGGSLRLSCAASGFTFSGFGMNWVRQAPGKGLEWVSYTSSSSRTIYYADSVKGRFTISRDNAQNSLYLQMNSLRDEDTAVYYCARDSSGWYDAFDIWGQGTMVTVSSASTKGPSVFPLAPSSKSTSGGTAALGCLVKDYFPEPVTVSWNSGALTSGVHTFPAVLQSSGLYSLSSVVTVPSSSLGTQTYICNVNHKPSNTKVDKKVEPKSCDKTHTCPPCPAPEAAGGPSVFLFPPKPKDTLMISRTPEVTCVVVDVSHEDPEVKFNWYVDGVEVHNAKTKPREEQYNSTYRVVSVLTVDHHDWLNGKEYKCKVSNKALPAPIEKTISKAKGQPREPQVYTLPPSREEMTKNQVSLTCLVKGFYPSDIAVEWESNGQPENNYKTTPPVLDSDGSFFLYSKLTVDKSRWQQGNVFSCSVMHEALHSHYTQKSLSLSPG

SEQ ID NO: 46 - protein, 447 aa, synthetic construct
EVQLVESGGGLVQPGGSLRLSCAASGFTFSGFGMNWVRQAPGKGLEWVSYTSSSSRTIYYADSVKGRFTISRDNAQNSLYLQMNSLRDEDTAVYYCARDSSGWYDAFDIWGQGTMVTVSSASTKGPSVFPLAPCSRSTSESTAALGCLVKDYFPEPVTVSWNSGALTSGVHTFPAVLQSSGLYSLSSVVTVPSSSLGTKTYTCNVDHKPSNTKVDKRVESKYGPPCPPCPAPEFLGGPSVFLFPPKPKDTLMISRTPEVTCVVVDVSQEDPEVQFNWYVDGVEVHNAKTKPREEQFNSTYRVVSVLTVLHQDWLNGKEYKCKVSNKGLPSSIEKTISKAKGQPREPQVYTLPPSQEEMTKNQVSLTCLVKGFYPSDIAVEWESNGQPENNYKTTPPVLDSDGSFFLYSRLTVDKSRWQEGNVFSCSVMHEALHNHYTQKSLSLSLGK

SEQ ID NO: 47 - protein, 446 aa, synthetic construct
EVQLVESGGGLVQPGGSLRLSCAASGFTFSGFGMNWVRQAPGKGLEWVSYTSSSSRTIYYADSVKGRFTISRDNAQNSLYLQMNSLRDEDTAVYYCARDSSGWYDAFDIWGQGTMVTVSSASTKGPSVFPLAPCSRSTSESTAALGCLVKDYFPEPVTVSWNSGALTSGVHTFPAVLQSSGLYSLSSVVTVPSSSLGTKTYTCNVDHKPSNTKVDKRVESKYGPPCPPCPAPEFLGGPSVFLFPPKPKDTLMISRTPEVTCVVVDVSQEDPEVQFNWYVDGVEVHNAKTKPREEQFNSTYRVVSVLTVLHQDWLNGKEYKCKVSNKGLPSSIEKTISKAKGQPREPQVYTLPPSQEEMTKNQVSLTCLVKGFYPSDIAVEWESNGQPENNYKTTPPVLDSDGSFFLYSRLTVDKSRWQEGNVFSCSVMHEALHNHYTQKSLSLSLG

SEQ ID NO: 48 - protein, 447 aa, synthetic construct
EVQLVESGGGLVQPGGSLRLSCAASGFTFSGFGMNWVRQAPGKGLEWVSYTSSSSRTIYYADSVKGRFTISRDNAQNSLYLQMNSLRDEDTAVYYCARDSSGWYDAFDIWGQGTMVTVSSASTKGPSVFPLAPCSRSTSESTAALGCLVKDYFPEPVTVSWNSGALTSGVHTFPAVLQSSGLYSLSSVVTVPSSSLGTKTYTCNVDHKPSNTKVDKRVESKYGPPCPPCPAPESTRGPSVFLFPPKPKDTLMISRTPEVTCVVVDVSQEDPEVQFNWYVDGVEVHNAKTKPREEQFNSTYRVVSVLTVLHQDWLNGKEYKCKVSNKGLPSSIEKTISKAKGQPREPQVYTLPPSQEEMTKNQVSLTCLVKGFYPSDIAVEWESNGQPENNYKTTPPVLDSDGSFFLYSRLTVDKSRWQEGNVFSCSVMHEALHNHYTQKSLSLSLGK

SEQ ID NO: 49 - protein, 446 aa, synthetic construct
EVQLVESGGGLVQPGGSLRLSCAASGFTFSGFGMNWVRQAPGKGLEWVSYTSSSSRTIYYADSVKGRFTISRDNAQNSLYLQMNSLRDEDTAVYYCARDSSGWYDAFDIWGQGTMVTVSSASTKGPSVFPLAPCSRSTSESTAALGCLVKDYFPEPVTVSWNSGALTSGVHTFPAVLQSSGLYSLSSVVTVPSSSLGTKTYTCNVDHKPSNTKVDKRVESKYGPPCPPCPAPESTRGPSVFLFPPKPKDTLMISRTPEVTCVVVDVSQEDPEVQFNWYVDGVEVHNAKTKPREEQFNSTYRVVSVLTVLHQDWLNGKEYKCKVSNKGLPSSIEKTISKAKGQPREPQVYTLPPSQEEMTKNQVSLTCLVKGFYPSDIAVEWESNGQPENNYKTTPPVLDSDGSFFLYSRLTVDKSRWQEGNVFSCSVMHEALHNHYTQKSLSLSLG

SEQ ID NO: 50 - protein, 447 aa, synthetic construct
EVQLVESGGGLVQPGGSLRLSCAASGFTFSGFGMNWVRQAPGKGLEWVSYTSSSSRTIYYADSVKGRFTISRDNAQNSLYLQMNSLRDEDTAVYYCARDSSGWYDAFDIWGQGTMVTVSSASTKGPSVFPLAPCSRSTSESTAALGCLVKDYFPEPVTVSWNSGALTSGVHTFPAVLQSSGLYSLSSVVTVPSSSLGTKTYTCNVDHKPSNTKVDKRVESKYGPPCPPCPAPEAAGGPSVFLFPPKPKDTLMISRTPEVTCVVVDVSQEDPEVQFNWYVDGVEVHNAKTKPREEQFNSTYRVVSVLTVLHQDWLNGKEYKCKVSNKGLPSSIEKTISKAKGQPREPQVYTLPPSQEEMTKNQVSLTCLVKGFYPSDIAVEWESNGQPENNYKTTPPVLDSDGSFFLYSRLTVDKSRWQEGNVFSCSVMHEALHNHYTQKSLSLSLGK

SEQ ID NO: 51 - protein, 446 aa, synthetic construct
EVQLVESGGGLVQPGGSLRLSCAASGFTFSGFGMNWVRQAPGKGLEWVSYTSSSSRTIYYADSVKGRFTISRDNAQNSLYLQMNSLRDEDTAVYYCARDSSGWYDAFDIWGQGTMVTVSSASTKGPSVFPLAPCSRSTSESTAALGCLVKDYFPEPVTVSWNSGALTSGVHTFPAVLQSSGLYSLSSVVTVPSSSLGTKTYTCNVDHKPSNTKVDKRVESKYGPPCPPCPAPEAAGGPSVFLFPPKPKDTLMISRTPEVTCVVVDVSQEDPEVQFNWYVDGVEVHNAKTKPREEQFNSTYRVVSVLTVLHQDWLNGKEYKCKVSNKGLPSSIEKTISKAKGQPREPQVYTLPPSQEEMTKNQVSLTCLVKGFYPSDIAVEWESNGQPENNYKTTPPVLDSDGSFFLYSRLTVDKSRWQEGNVFSCSVMHEALHNHYTQKSLSLSLG

SEQ ID NO: 52 - protein, 447 aa, synthetic construct
EVQLVESGGGLVQPGGSLRLSCAASGFTFSGFGMNWVRQAPGKGLEWVSYTSSSSRTIYYADSVKGRFTISRDNAQNSLYLQMNSLRDEDTAVYYCARDSSGWYDAFDIWGQGTMVTVSSASTKGPSVFPLAPCSRSTSESTAALGCLVKDYFPEPVTVSWNSGALTSGVHTFPAVLQSSGLYSLSSVVTVPSSSLGTKTYTCNVDHKPSNTKVDKRVESKYGPPCPPCPAPEFLGGPSVFLFPPKPKDTLYITREPEVTCVVVDVSQEDPEVQFNWYVDGVEVHNAKTKPREEQFNSTYRVVSVLTVLHQDWLNGKEYKCKVSNKGLPSSIEKTISKAKGQPREPQVYTLPPSQEEMTKNQVSLTCLVKGFYPSDIAVEWESNGQPENNYKTTPPVLDSDGSFFLYSRLTVDKSRWQEGNVFSCSVMHEALHNHYTQKSLSLSLGK

SEQ ID NO: 53 - protein, 446 aa, synthetic construct
EVQLVESGGGLVQPGGSLRLSCAASGFTFSGFGMNWVRQAPGKGLEWVSYTSSSSRTIYYADSVKGRFTISRDNAQNSLYLQMNSLRDEDTAVYYCARDSSGWYDAFDIWGQGTMVTVSSASTKGPSVFPLAPCSRSTSESTAALGCLVKDYFPEPVTVSWNSGALTSGVHTFPAVLQSSGLYSLSSVVTVPSSSLGTKTYTCNVDHKPSNTKVDKRVESKYGPPCPPCPAPEFLGGPSVFLFPPKPKDTLYITREPEVTCVVVDVSQEDPEVQFNWYVDGVEVHNAKTKPREEQFNSTYRVVSVLTVLHQDWLNGKEYKCKVSNKGLPSSIEKTISKAKGQPREPQVYTLPPSQEEMTKNQVSLTCLVKGFYPSDIAVEWESNGQPENNYKTTPPVLDSDGSFFLYSRLTVDKSRWQEGNVFSCSVMHEALHNHYTQKSLSLSLG

SEQ ID NO: 54 - protein, 447 aa, synthetic construct
EVQLVESGGGLVQPGGSLRLSCAASGFTFSGFGMNWVRQAPGKGLEWVSYTSSSSRTIYYADSVKGRFTISRDNAQNSLYLQMNSLRDEDTAVYYCARDSSGWYDAFDIWGQGTMVTVSSASTKGPSVFPLAPCSRSTSESTAALGCLVKDYFPEPVTVSWNSGALTSGVHTFPAVLQSSGLYSLSSVVTVPSSSLGTKTYTCNVDHKPSNTKVDKRVESKYGPPCPPCPAPESTRGPSVFLFPPKPKDTLYITREPEVTCVVVDVSQEDPEVQFNWYVDGVEVHNAKTKPREEQFNSTYRVVSVLTVLHQDWLNGKEYKCKVSNKGLPSSIEKTISKAKGQPREPQVYTLPPSQEEMTKNQVSLTCLVKGFYPSDIAVEWESNGQPENNYKTTPPVLDSDGSFFLYSRLTVDKSRWQEGNVFSCSVMHEALHNHYTQKSLSLSLGK

SEQ ID NO: 55 - protein, 446 aa, synthetic construct
EVQLVESGGGLVQPGGSLRLSCAASGFTFSGFGMNWVRQAPGKGLEWVSYTSSSSRTIYYADSVKGRFTISRDNAQNSLYLQMNSLRDEDTAVYYCARDSSGWYDAFDIWGQGTMVTVSSASTKGPSVFPLAPCSRSTSESTAALGCLVKDYFPEPVTVSWNSGALTSGVHTFPAVLQSSGLYSLSSVVTVPSSSLGTKTYTCNVDHKPSNTKVDKRVESKYGPPCPPCPAPESTRGPSVFLFPPKPKDTLYITREPEVTCVVVDVSQEDPEVQFNWYVDGVEVHNAKTKPREEQFNSTYRVVSVLTVLHQDWLNGKEYKCKVSNKGLPSSIEKTISKAKGQPREPQVYTLPPSQEEMTKNQVSLTCLVKGFYPSDIAVEWESNGQPENNYKTTPPVLDSDGSFFLYSRLTVDKSRWQEGNVFSCSVMHEALHNHYTQKSLSLSLG

SEQ ID NO: 56 - protein, 447 aa, synthetic construct
EVQLVESGGGLVQPGGSLRLSCAASGFTFSGFGMNWVRQAPGKGLEWVSYTSSSSRTIYYADSVKGRFTISRDNAQNSLYLQMNSLRDEDTAVYYCARDSSGWYDAFDIWGQGTMVTVSSASTKGPSVFPLAPCSRSTSESTAALGCLVKDYFPEPVTVSWNSGALTSGVHTFPAVLQSSGLYSLSSVVTVPSSSLGTKTYTCNVDHKPSNTKVDKRVESKYGPPCPPCPAPEAAGGPSVFLFPPKPKDTLYITREPEVTCVVVDVSQEDPEVQFNWYVDGVEVHNAKTKPREEQFNSTYRVVSVLTVLHQDWLNGKEYKCKVSNKGLPSSIEKTISKAKGQPREPQVYTLPPSQEEMTKNQVSLTCLVKGFYPSDIAVEWESNGQPENNYKTTPPVLDSDGSFFLYSRLTVDKSRWQEGNVFSCSVMHEALHNHYTQKSLSLSLGK

SEQ ID NO: 57 - protein, 446 aa, synthetic construct
EVQLVESGGGLVQPGGSLRLSCAASGFTFSGFGMNWVRQAPGKGLEWVSYTSSSSRTIYYADSVKGRFTISRDNAQNSLYLQMNSLRDEDTAVYYCARDSSGWYDAFDIWGQGTMVTVSSASTKGPSVFPLAPCSRSTSESTAALGCLVKDYFPEPVTVSWNSGALTSGVHTFPAVLQSSGLYSLSSVVTVPSSSLGTKTYTCNVDHKPSNTKVDKRVESKYGPPCPPCPAPEAAGGPSVFLFPPKPKDTLYITREPEVTCVVVDVSQEDPEVQFNWYVDGVEVHNAKTKPREEQFNSTYRVVSVLTVLHQDWLNGKEYKCKVSNKGLPSSIEKTISKAKGQPREPQVYTLPPSQEEMTKNQVSLTCLVKGFYPSDIAVEWESNGQPENNYKTTPPVLDSDGSFFLYSRLTVDKSRWQEGNVFSCSVMHEALHNHYTQKSLSLSLG

SEQ ID NO: 58 - protein, 447 aa, synthetic construct
EVQLVESGGGLVQPGGSLRLSCAASGFTFSGFGMNWVRQAPGKGLEWVSYTSSSSRTIYYADSVKGRFTISRDNAQNSLYLQMNSLRDEDTAVYYCARDSSGWYDAFDIWGQGTMVTVSSASTKGPSVFPLAPCSRSTSESTAALGCLVKDYFPEPVTVSWNSGALTSGVHTFPAVLQSSGLYSLSSVVTVPSSSLGTKTYTCNVDHKPSNTKVDKRVESKYGPPCPPCPAPEFLGGPSVFLFPPKPKDTLMISRTPEVTCVVVDVSQEDPEVQFNWYVDGVEVHNAKTKPREEQFNSTYRVVSVLTVLHRDWLNGKEYKCKVSNKGLPSSIEKTISKAKGQPREPQVYTLPPSQEEMTKNQVSLTCLVKGFYPSDIAVEWESNGQPENNYKTTPPVLDSDGSFFLYSRLTVDKSRWQEGNVFSCSVEHEALHWHYTQKSLSLSLGK

SEQ ID NO: 59 - protein, 446 aa, synthetic construct
EVQLVESGGGLVQPGGSLRLSCAASGFTFSGFGMNWVRQAPGKGLEWVSYTSSSSRTIYYADSVKGRFTISRDNAQNSLYLQMNSLRDEDTAVYYCARDSSGWYDAFDIWGQGTMVTVSSASTKGPSVFPLAPCSRSTSESTAALGCLVKDYFPEPVTVSWNSGALTSGVHTFPAVLQSSGLYSLSSVVTVPSSSLGTKTYTCNVDHKPSNTKVDKRVESKYGPPCPPCPAPEFLGGPSVFLFPPKPKDTLMISRTPEVTCVVVDVSQEDPEVQFNWYVDGVEVHNAKTKPREEQFNSTYRVVSVLTVLHRDWLNGKEYKCKVSNKGLPSSIEKTISKAKGQPREPQVYTLPPSQEEMTKNQVSLTCLVKGFYPSDIAVEWESNGQPENNYKTTPPVLDSDGSFFLYSRLTVDKSRWQEGNVFSCSVEHEALHWHYTQKSLSLSLG

SEQ ID NO: 60 - protein, 447 aa, synthetic construct
EVQLVESGGGLVQPGGSLRLSCAASGFTFSGFGMNWVRQAPGKGLEWVSYTSSSSRTIYYADSVKGRFTISRDNAQNSLYLQMNSLRDEDTAVYYCARDSSGWYDAFDIWGQGTMVTVSSASTKGPSVFPLAPCSRSTSESTAALGCLVKDYFPEPVTVSWNSGALTSGVHTFPAVLQSSGLYSLSSVVTVPSSSLGTKTYTCNVDHKPSNTKVDKRVESKYGPPCPPCPAPESTRGPSVFLFPPKPKDTLMISRTPEVTCVVVDVSQEDPEVQFNWYVDGVEVHNAKTKPREEQFNSTYRVVSVLTVLHRDWLNGKEYKCKVSNKGLPSSIEKTISKAKGQPREPQVYTLPPSQEEMTKNQVSLTCLVKGFYPSDIAVEWESNGQPENNYKTTPPVLDSDGSFFLYSRLTVDKSRWQEGNVFSCSVEHEALHWHYTQKSLSLSLGK

SEQ ID NO: 61 - protein, 446 aa, synthetic construct
EVQLVESGGGLVQPGGSLRLSCAASGFTFSGFGMNWVRQAPGKGLEWVSYTSSSSRTIYYADSVKGRFTISRDNAQNSLYLQMNSLRDEDTAVYYCARDSSGWYDAFDIWGQGTMVTVSSASTKGPSVFPLAPCSRSTSESTAALGCLVKDYFPEPVTVSWNSGALTSGVHTFPAVLQSSGLYSLSSVVTVPSSSLGTKTYTCNVDHKPSNTKVDKRVESKYGPPCPPCPAPESTRGPSVFLFPPKPKDTLMISRTPEVTCVVVDVSQEDPEVQFNWYVDGVEVHNAKTKPREEQFNSTYRVVSVLTVLHRDWLNGKEYKCKVSNKGLPSSIEKTISKAKGQPREPQVYTLPPSQEEMTKNQVSLTCLVKGFYPSDIAVEWESNGQPENNYKTTPPVLDSDGSFFLYSRLTVDKSRWQEGNVFSCSVEHEALHWHYTQKSLSLSLG

SEQ ID NO: 62 - protein, 447 aa, synthetic construct
EVQLVESGGGLVQPGGSLRLSCAASGFTFSGFGMNWVRQAPGKGLEWVSYTSSSSRTIYYADSVKGRFTISRDNAQNSLYLQMNSLRDEDTAVYYCARDSSGWYDAFDIWGQGTMVTVSSASTKGPSVFPLAPCSRSTSESTAALGCLVKDYFPEPVTVSWNSGALTSGVHTFPAVLQSSGLYSLSSVVTVPSSSLGTKTYTCNVDHKPSNTKVDKRVESKYGPPCPPCPAPEAAGGPSVFLFPPKPKDTLMISRTPEVTCVVVDVSQEDPEVQFNWYVDGVEVHNAKTKPREEQFNSTYRVVSVLTVLHRDWLNGKEYKCKVSNKGLPSSIEKTISKAKGQPREPQVYTLPPSQEEMTKNQVSLTCLVKGFYPSDIAVEWESNGQPENNYKTTPPVLDSDGSFFLYSRLTVDKSRWQEGNVFSCSVEHEALHWHYTQKSLSLSLGK

SEQ ID NO: 63 - protein, 446 aa, synthetic construct
EVQLVESGGGLVQPGGSLRLSCAASGFTFSGFGMNWVRQAPGKGLEWVSYTSSSSRTIYYADSVKGRFTISRDNAQNSLYLQMNSLRDEDTAVYYCARDSSGWYDAFDIWGQGTMVTVSSASTKGPSVFPLAPCSRSTSESTAALGCLVKDYFPEPVTVSWNSGALTSGVHTFPAVLQSSGLYSLSSVVTVPSSSLGTKTYTCNVDHKPSNTKVDKRVESKYGPPCPPCPAPEAAGGPSVFLFPPKPKDTLMISRTPEVTCVVVDVSQEDPEVQFNWYVDGVEVHNAKTKPREEQFNSTYRVVSVLTVLHRDWLNGKEYKCKVSNKGLPSSIEKTISKAKGQPREPQVYTLPPSQEEMTKNQVSLTCLVKGFYPSDIAVEWESNGQPENNYKTTPPVLDSDGSFFLYSRLTVDKSRWQEGNVFSCSVEHEALHWHYTQKSLSLSLG

SEQ ID NO: 64 - protein, 447 aa, synthetic construct
EVQLVESGGGLVQPGGSLRLSCAASGFTFSGFGMNWVRQAPGKGLEWVSYTSSSSRTIYYADSVKGRFTISRDNAQNSLYLQMNSLRDEDTAVYYCARDSSGWYDAFDIWGQGTMVTVSSASTKGPSVFPLAPCSRSTSESTAALGCLVKDYFPEPVTVSWNSGALTSGVHTFPAVLQSSGLYSLSSVVTVPSSSLGTKTYTCNVDHKPSNTKVDKRVESKYGPPCPPCPAPEFLGGPSVFLFPPKPKDTLMISRTPEVTCVVVDVSQEDPEVQFNWYVDGVEVHNAKTKPREEQFNSTYRVVSVLTVLHQDWLNGKEYKCKVSNKGLPSSIEKTISKAKGQPREPQVYTLPPSQEEMTKNQVSLTCLVKGFYPSDIAVEWESNGQPENNYKTTPPVLDSDGSFFLYSRLTVDKSRWQEGNVFSCSVLHEALHSHYTQKSLSLSLGK

SEQ ID NO: 65 - protein, 446 aa, synthetic construct
EVQLVESGGGLVQPGGSLRLSCAASGFTFSGFGMNWVRQAPGKGLEWVSYTSSSSRTIYYADSVKGRFTISRDNAQNSLYLQMNSLRDEDTAVYYCARDSSGWYDAFDIWGQGTMVTVSSASTKGPSVFPLAPCSRSTSESTAALGCLVKDYFPEPVTVSWNSGALTSGVHTFPAVLQSSGLYSLSSVVTVPSSSLGTKTYTCNVDHKPSNTKVDKRVESKYGPPCPPCPAPEFLGGPSVFLFPPKPKDTLMISRTPEVTCVVVDVSQEDPEVQFNWYVDGVEVHNAKTKPREEQFNSTYRVVSVLTVLHQDWLNGKEYKCKVSNKGLPSSIEKTISKAKGQPREPQVYTLPPSQEEMTKNQVSLTCLVKGFYPSDIAVEWESNGQPENNYKTTPPVLDSDGSFFLYSRLTVDKSRWQEGNVFSCSVLHEALHSHYTQKSLSLSLG

SEQ ID NO: 66 - protein, 447 aa, synthetic construct
EVQLVESGGGLVQPGGSLRLSCAASGFTFSGFGMNWVRQAPGKGLEWVSYTSSSSRTIYYADSVKGRFTISRDNAQNSLYLQMNSLRDEDTAVYYCARDSSGWYDAFDIWGQGTMVTVSSASTKGPSVFPLAPCSRSTSESTAALGCLVKDYFPEPVTVSWNSGALTSGVHTFPAVLQSSGLYSLSSVVTVPSSSLGTKTYTCNVDHKPSNTKVDKRVESKYGPPCPPCPAPESTRGPSVFLFPPKPKDTLMISRTPEVTCVVVDVSQEDPEVQFNWYVDGVEVHNAKTKPREEQFNSTYRVVSVLTVLHQDWLNGKEYKCKVSNKGLPSSIEKTISKAKGQPREPQVYTLPPSQEEMTKNQVSLTCLVKGFYPSDIAVEWESNGQPENNYKTTPPVLDSDGSFFLYSRLTVDKSRWQEGNVFSCSVLHEALHSHYTQKSLSLSLGK

SEQ ID NO: 67 - protein, 446 aa, synthetic construct
EVQLVESGGGLVQPGGSLRLSCAASGFTFSGFGMNWVRQAPGKGLEWVSYTSSSSRTIYYADSVKGRFTISRDNAQNSLYLQMNSLRDEDTAVYYCARDSSGWYDAFDIWGQGTMVTVSSASTKGPSVFPLAPCSRSTSESTAALGCLVKDYFPEPVTVSWNSGALTSGVHTFPAVLQSSGLYSLSSVVTVPSSSLGTKTYTCNVDHKPSNTKVDKRVESKYGPPCPPCPAPESTRGPSVFLFPPKPKDTLMISRTPEVTCVVVDVSQEDPEVQFNWYVDGVEVHNAKTKPREEQFNSTYRVVSVLTVLHQDWLNGKEYKCKVSNKGLPSSIEKTISKAKGQPREPQVYTLPPSQEEMTKNQVSLTCLVKGFYPSDIAVEWESNGQPENNYKTTPPVLDSDGSFFLYSRLTVDKSRWQEGNVFSCSVLHEALHSHYTQKSLSLSLG

SEQ ID NO: 68 - protein, 447 aa, synthetic construct
EVQLVESGGGLVQPGGSLRLSCAASGFTFSGFGMNWVRQAPGKGLEWVSYTSSSSRTIYYADSVKGRFTISRDNAQNSLYLQMNSLRDEDTAVYYCARDSSGWYDAFDIWGQGTMVTVSSASTKGPSVFPLAPCSRSTSESTAALGCLVKDYFPEPVTVSWNSGALTSGVHTFPAVLQSSGLYSLSSVVTVPSSSLGTKTYTCNVDHKPSNTKVDKRVESKYGPPCPPCPAPEAAGGPSVFLFPPKPKDTLMISRTPEVTCVVVDVSQEDPEVQFNWYVDGVEVHNAKTKPREEQFNSTYRVVSVLTVLHQDWLNGKEYKCKVSNKGLPSSIEKTISKAKGQPREPQVYTLPPSQEEMTKNQVSLTCLVKGFYPSDIAVEWESNGQPENNYKTTPPVLDSDGSFFLYSRLTVDKSRWQEGNVFSCSVLHEALHSHYTQKSLSLSLGK

SEQ ID NO: 69 - protein, 446 aa, synthetic construct
EVQLVESGGGLVQPGGSLRLSCAASGFTFSGFGMNWVRQAPGKGLEWVSYTSSSSRTIYYADSVKGRFTISRDNAQNSLYLQMNSLRDEDTAVYYCARDSSGWYDAFDIWGQGTMVTVSSASTKGPSVFPLAPCSRSTSESTAALGCLVKDYFPEPVTVSWNSGALTSGVHTFPAVLQSSGLYSLSSVVTVPSSSLGTKTYTCNVDHKPSNTKVDKRVESKYGPPCPPCPAPEAAGGPSVFLFPPKPKDTLMISRTPEVTCVVVDVSQEDPEVQFNWYVDGVEVHNAKTKPREEQFNSTYRVVSVLTVLHQDWLNGKEYKCKVSNKGLPSSIEKTISKAKGQPREPQVYTLPPSQEEMTKNQVSLTCLVKGFYPSDIAVEWESNGQPENNYKTTPPVLDSDGSFFLYSRLTVDKSRWQEGNVFSCSVLHEALHSHYTQKSLSLSLG

SEQ ID NO: 70 - protein, 447 aa, synthetic construct
EVQLVESGGGLVQPGGSLRLSCAASGFTFSGFGMNWVRQAPGKGLEWVSYTSSSSRTIYYADSVKGRFTISRDNAQNSLYLQMNSLRDEDTAVYYCARDSSGWYDAFDIWGQGTMVTVSSASTKGPSVFPLAPCSRSTSESTAALGCLVKDYFPEPVTVSWNSGALTSGVHTFPAVLQSSGLYSLSSVVTVPSSSLGTKTYTCNVDHKPSNTKVDKRVESKYGPPCPPCPAPEFLGGPSVFLFPPKPKDQLMISRTPEVTCVVVDVSQEDPEVQFNWYVDGVEVHNAKTKPREEQFNSTYRVVSVLTVLHQDWLNGKEYKCKVSNKGLPSSIEKTISKAKGQPREPQVYTLPPSQEEMTKNQVSLTCLVKGFYPSDIAVEWESNGQPENNYKTTPPVLDSDGSFFLYSRLTVDKSRWQEGNVFSCSVLHEALHNHYTQKSLSLSLGK

SEQ ID NO: 71 - protein, 446 aa, synthetic construct
EVQLVESGGGLVQPGGSLRLSCAASGFTFSGFGMNWVRQAPGKGLEWVSYTSSSSRTIYYADSVKGRFTISRDNAQNSLYLQMNSLRDEDTAVYYCARDSSGWYDAFDIWGQGTMVTVSSASTKGPSVFPLAPCSRSTSESTAALGCLVKDYFPEPVTVSWNSGALTSGVHTFPAVLQSSGLYSLSSVVTVPSSSLGTKTYTCNVDHKPSNTKVDKRVESKYGPPCPPCPAPEFLGGPSVFLFPPKPKDQLMISRTPEVTCVVVDVSQEDPEVQFNWYVDGVEVHNAKTKPREEQFNSTYRVVSVLTVLHQDWLNGKEYKCKVSNKGLPSSIEKTISKAKGQPREPQVYTLPPSQEEMTKNQVSLTCLVKGFYPSDIAVEWESNGQPENNYKTTPPVLDSDGSFFLYSRLTVDKSRWQEGNVFSCSVLHEALHNHYTQKSLSLSLG

SEQ ID NO: 72 - protein, 447 aa, synthetic construct
EVQLVESGGGLVQPGGSLRLSCAASGFTFSGFGMNWVRQAPGKGLEWVSYTSSSSRTIYYADSVKGRFTISRDNAQNSLYLQMNSLRDEDTAVYYCARDSSGWYDAFDIWGQGTMVTVSSASTKGPSVFPLAPCSRSTSESTAALGCLVKDYFPEPVTVSWNSGALTSGVHTFPAVLQSSGLYSLSSVVTVPSSSLGTKTYTCNVDHKPSNTKVDKRVESKYGPPCPPCPAPESTRGPSVFLFPPKPKDQLMISRTPEVTCVVVDVSQEDPEVQFNWYVDGVEVHNAKTKPREEQFNSTYRVVSVLTVLHQDWLNGKEYKCKVSNKGLPSSIEKTISKAKGQPREPQVYTLPPSQEEMTKNQVSLTCLVKGFYPSDIAVEWESNGQPENNYKTTPPVLDSDGSFFLYSRLTVDKSRWQEGNVFSCSVLHEALHNHYTQKSLSLSLGK

SEQ ID NO: 73 - protein, 446 aa, synthetic construct
EVQLVESGGGLVQPGGSLRLSCAASGFTFSGFGMNWVRQAPGKGLEWVSYTSSSSRTIYYADSVKGRFTISRDNAQNSLYLQMNSLRDEDTAVYYCARDSSGWYDAFDIWGQGTMVTVSSASTKGPSVFPLAPCSRSTSESTAALGCLVKDYFPEPVTVSWNSGALTSGVHTFPAVLQSSGLYSLSSVVTVPSSSLGTKTYTCNVDHKPSNTKVDKRVESKYGPPCPPCPAPESTRGPSVFLFPPKPKDQLMISRTPEVTCVVVDVSQEDPEVQFNWYVDGVEVHNAKTKPREEQFNSTYRVVSVLTVLHQDWLNGKEYKCKVSNKGLPSSIEKTISKAKGQPREPQVYTLPPSQEEMTKNQVSLTCLVKGFYPSDIAVEWESNGQPENNYKTTPPVLDSDGSFFLYSRLTVDKSRWQEGNVFSCSVLHEALHNHYTQKSLSLSLG

SEQ ID NO: 74 - protein, 447 aa, synthetic construct
EVQLVESGGGLVQPGGSLRLSCAASGFTFSGFGMNWVRQAPGKGLEWVSYTSSSSRTIYYADSVKGRFTISRDNAQNSLYLQMNSLRDEDTAVYYCARDSSGWYDAFDIWGQGTMVTVSSASTKGPSVFPLAPCSRSTSESTAALGCLVKDYFPEPVTVSWNSGALTSGVHTFPAVLQSSGLYSLSSVVTVPSSSLGTKTYTCNVDHKPSNTKVDKRVESKYGPPCPPCPAPEAAGGPSVFLFPPKPKDQLMISRTPEVTCVVVDVSQEDPEVQFNWYVDGVEVHNAKTKPREEQFNSTYRVVSVLTVLHQDWLNGKEYKCKVSNKGLPSSIEKTISKAKGQPREPQVYTLPPSQEEMTKNQVSLTCLVKGFYPSDIAVEWESNGQPENNYKTTPPVLDSDGSFFLYSRLTVDKSRWQEGNVFSCSVLHEALHNHYTQKSLSLSLGK

SEQ ID NO: 75 - protein, 446 aa, synthetic construct
EVQLVESGGGLVQPGGSLRLSCAASGFTFSGFGMNWVRQAPGKGLEWVSYTSSSSRTIYYADSVKGRFTISRDNAQNSLYLQMNSLRDEDTAVYYCARDSSGWYDAFDIWGQGTMVTVSSASTKGPSVFPLAPCSRSTSESTAALGCLVKDYFPEPVTVSWNSGALTSGVHTFPAVLQSSGLYSLSSVVTVPSSSLGTKTYTCNVDHKPSNTKVDKRVESKYGPPCPPCPAPEAAGGPSVFLFPPKPKDQLMISRTPEVTCVVVDVSQEDPEVQFNWYVDGVEVHNAKTKPREEQFNSTYRVVSVLTVLHQDWLNGKEYKCKVSNKGLPSSIEKTISKAKGQPREPQVYTLPPSQEEMTKNQVSLTCLVKGFYPSDIAVEWESNGQPENNYKTTPPVLDSDGSFFLYSRLTVDKSRWQEGNVFSCSVLHEALHNHYTQKSLSLSLG

SEQ ID NO: 76 - protein, 447 aa, synthetic construct
EVQLVESGGGLVQPGGSLRLSCAASGFTFSGFGMNWVRQAPGKGLEWVSYTSSSSRTIYYADSVKGRFTISRDNAQNSLYLQMNSLRDEDTAVYYCARDSSGWYDAFDIWGQGTMVTVSSASTKGPSVFPLAPCSRSTSESTAALGCLVKDYFPEPVTVSWNSGALTSGVHTFPAVLQSSGLYSLSSVVTVPSSSLGTKTYTCNVDHKPSNTKVDKRVESKYGPPCPPCPAPEFLGGPSVFLFPPKPKDTLMISRTPEVTCVVVDVSQEDPEVQFNWYVDGVEVHNAKTKPREEQFNSTYRVVSVLTVDHHDWLNGKEYKCKVSNKGLPSSIEKTISKAKGQPREPQVYTLPPSQEEMTKNQVSLTCLVKGFYPSDIAVEWESNGQPENNYKTTPPVLDSDGSFFLYSRLTVDKSRWQEGNVFSCSVMHEALHSHYTQKSLSLSLGK

SEQ ID NO: 77 - protein, 446 aa, synthetic construct
EVQLVESGGGLVQPGGSLRLSCAASGFTFSGFGMNWVRQAPGKGLEWVSYTSSSSRTIYYADSVKGRFTISRDNAQNSLYLQMNSLRDEDTAVYYCARDSSGWYDAFDIWGQGTMVTVSSASTKGPSVFPLAPCSRSTSESTAALGCLVKDYFPEPVTVSWNSGALTSGVHTFPAVLQSSGLYSLSSVVTVPSSSLGTKTYTCNVDHKPSNTKVDKRVESKYGPPCPPCPAPEFLGGPSVFLFPPKPKDTLMISRTPEVTCVVVDVSQEDPEVQFNWYVDGVEVHNAKTKPREEQFNSTYRVVSVLTVDHHDWLNGKEYKCKVSNKGLPSSIEKTISKAKGQPREPQVYTLPPSQEEMTKNQVSLTCLVKGFYPSDIAVEWESNGQPENNYKTTPPVLDSDGSFFLYSRLTVDKSRWQEGNVFSCSVMHEALHSHYTQKSLSLSLG

SEQ ID NO: 78 - protein, 447 aa, synthetic construct
EVQLVESGGGLVQPGGSLRLSCAASGFTFSGFGMNWVRQAPGKGLEWVSYTSSSSRTIYYADSVKGRFTISRDNAQNSLYLQMNSLRDEDTAVYYCARDSSGWYDAFDIWGQGTMVTVSSASTKGPSVFPLAPCSRSTSESTAALGCLVKDYFPEPVTVSWNSGALTSGVHTFPAVLQSSGLYSLSSVVTVPSSSLGTKTYTCNVDHKPSNTKVDKRVESKYGPPCPPCPAPESTRGPSVFLFPPKPKDTLMISRTPEVTCVVVDVSQEDPEVQFNWYVDGVEVHNAKTKPREEQFNSTYRVVSVLTVDHHDWLNGKEYKCKVSNKGLPSSIEKTISKAKGQPREPQVYTLPPSQEEMTKNQVSLTCLVKGFYPSDIAVEWESNGQPENNYKTTPPVLDSDGSFFLYSRLTVDKSRWQEGNVFSCSVMHEALHSHYTQKSLSLSLGK

SEQ ID NO: 79 - protein, 446 aa, synthetic construct
EVQLVESGGGLVQPGGSLRLSCAASGFTFSGFGMNWVRQAPGKGLEWVSYTSSSSRTIYYADSVKGRFTISRDNAQNSLYLQMNSLRDEDTAVYYCARDSSGWYDAFDIWGQGTMVTVSSASTKGPSVFPLAPCSRSTSESTAALGCLVKDYFPEPVTVSWNSGALTSGVHTFPAVLQSSGLYSLSSVVTVPSSSLGTKTYTCNVDHKPSNTKVDKRVESKYGPPCPPCPAPESTRGPSVFLFPPKPKDTLMISRTPEVTCVVVDVSQEDPEVQFNWYVDGVEVHNAKTKPREEQFNSTYRVVSVLTVDHHDWLNGKEYKCKVSNKGLPSSIEKTISKAKGQPREPQVYTLPPSQEEMTKNQVSLTCLVKGFYPSDIAVEWESNGQPENNYKTTPPVLDSDGSFFLYSRLTVDKSRWQEGNVFSCSVMHEALHSHYTQKSLSLSLG

SEQ ID NO: 80 - protein, 447 aa, synthetic construct
EVQLVESGGGLVQPGGSLRLSCAASGFTFSGFGMNWVRQAPGKGLEWVSYTSSSSRTIYYADSVKGRFTISRDNAQNSLYLQMNSLRDEDTAVYYCARDSSGWYDAFDIWGQGTMVTVSSASTKGPSVFPLAPCSRSTSESTAALGCLVKDYFPEPVTVSWNSGALTSGVHTFPAVLQSSGLYSLSSVVTVPSSSLGTKTYTCNVDHKPSNTKVDKRVESKYGPPCPPCPAPEAAGGPSVFLFPPKPKDTLMISRTPEVTCVVVDVSQEDPEVQFNWYVDGVEVHNAKTKPREEQFNSTYRVVSVLTVDHHDWLNGKEYKCKVSNKGLPSSIEKTISKAKGQPREPQVYTLPPSQEEMTKNQVSLTCLVKGFYPSDIAVEWESNGQPENNYKTTPPVLDSDGSFFLYSRLTVDKSRWQEGNVFSCSVMHEALHSHYTQKSLSLSLGK

SEQ ID NO: 81 - protein, 446 aa, synthetic construct
EVQLVESGGGLVQPGGSLRLSCAASGFTFSGFGMNWVRQAPGKGLEWVSYTSSSSRTIYYADSVKGRFTISRDNAQNSLYLQMNSLRDEDTAVYYCARDSSGWYDAFDIWGQGTMVTVSSASTKGPSVFPLAPCSRSTSESTAALGCLVKDYFPEPVTVSWNSGALTSGVHTFPAVLQSSGLYSLSSVVTVPSSSLGTKTYTCNVDHKPSNTKVDKRVESKYGPPCPPCPAPEAAGGPSVFLFPPKPKDTLMISRTPEVTCVVVDVSQEDPEVQFNWYVDGVEVHNAKTKPREEQFNSTYRVVSVLTVDHHDWLNGKEYKCKVSNKGLPSSIEKTISKAKGQPREPQVYTLPPSQEEMTKNQVSLTCLVKGFYPSDIAVEWESNGQPENNYKTTPPVLDSDGSFFLYSRLTVDKSRWQEGNVFSCSVMHEALHSHYTQKSLSLSLG

SEQ ID NO: 82 - protein, 447 aa, synthetic construct
EVQLVESGGGLVQPGGSLRLSCAASGFTFSGFGMNWVRQAPGKGLEWVSYTSSSSRTIYYADSVKGRFTISRDNAQNSLYLQMNSLRDEDTAVYYCARDSSGWYDAFDIWGQGTMVTVSSASTKGPSVFPLAPCSRSTSESTAALGCLVKDYFPEPVTVSWNSGALTSGVHTFPAVLQSSGLYSLSSVVTVPSSSLGTKTYTCNVDHKPSNTKVDKRVESKYGPPCPSCPAPEFLGGPSVFLFPPKPKDTLMISRTPEVTCVVVDVSQEDPEVQFNWYVDGVEVHNAKTKPREEQFNSTYRVVSVLTVLHQDWLNGKEYKCKVSNKGLPSSIEKTISKAKGQPREPQVYTLPPSQEEMTKNQVSLTCLVKGFYPSDIAVEWESNGQPENNYKTTPPVLDSDGSFFLYSRLTVDKSRWQEGNVFSCSVMHEALHNHYTQKSLSLSLGK

SEQ ID NO: 83 - protein, 446 aa, synthetic construct
EVQLVESGGGLVQPGGSLRLSCAASGFTFSGFGMNWVRQAPGKGLEWVSYTSSSSRTIYYADSVKGRFTISRDNAQNSLYLQMNSLRDEDTAVYYCARDSSGWYDAFDIWGQGTMVTVSSASTKGPSVFPLAPCSRSTSESTAALGCLVKDYFPEPVTVSWNSGALTSGVHTFPAVLQSSGLYSLSSVVTVPSSSLGTKTYTCNVDHKPSNTKVDKRVESKYGPPCPSCPAPEFLGGPSVFLFPPKPKDTLMISRTPEVTCVVVDVSQEDPEVQFNWYVDGVEVHNAKTKPREEQFNSTYRVVSVLTVLHQDWLNGKEYKCKVSNKGLPSSIEKTISKAKGQPREPQVYTLPPSQEEMTKNQVSLTCLVKGFYPSDIAVEWESNGQPENNYKTTPPVLDSDGSFFLYSRLTVDKSRWQEGNVFSCSVMHEALHNHYTQKSLSLSLG

SEQ ID NO: 84 - protein, 447 aa, synthetic construct
EVQLVESGGGLVQPGGSLRLSCAASGFTFSGFGMNWVRQAPGKGLEWVSYTSSSSRTIYYADSVKGRFTISRDNAQNSLYLQMNSLRDEDTAVYYCARDSSGWYDAFDIWGQGTMVTVSSASTKGPSVFPLAPCSRSTSESTAALGCLVKDYFPEPVTVSWNSGALTSGVHTFPAVLQSSGLYSLSSVVTVPSSSLGTKTYTCNVDHKPSNTKVDKRVESKYGPPCPSCPAPESTRGPSVFLFPPKPKDTLMISRTPEVTCVVVDVSQEDPEVQFNWYVDGVEVHNAKTKPREEQFNSTYRVVSVLTVLHQDWLNGKEYKCKVSNKGLPSSIEKTISKAKGQPREPQVYTLPPSQEEMTKNQVSLTCLVKGFYPSDIAVEWESNGQPENNYKTTPPVLDSDGSFFLYSRLTVDKSRWQEGNVFSCSVMHEALHNHYTQKSLSLSLGK

SEQ ID NO: 85 - protein, 446 aa, synthetic construct
EVQLVESGGGLVQPGGSLRLSCAASGFTFSGFGMNWVRQAPGKGLEWVSYTSSSSRTIYYADSVKGRFTISRDNAQNSLYLQMNSLRDEDTAVYYCARDSSGWYDAFDIWGQGTMVTVSSASTKGPSVFPLAPCSRSTSESTAALGCLVKDYFPEPVTVSWNSGALTSGVHTFPAVLQSSGLYSLSSVVTVPSSSLGTKTYTCNVDHKPSNTKVDKRVESKYGPPCPSCPAPESTRGPSVFLFPPKPKDTLMISRTPEVTCVVVDVSQEDPEVQFNWYVDGVEVHNAKTKPREEQFNSTYRVVSVLTVLHQDWLNGKEYKCKVSNKGLPSSIEKTISKAKGQPREPQVYTLPPSQEEMTKNQVSLTCLVKGFYPSDIAVEWESNGQPENNYKTTPPVLDSDGSFFLYSRLTVDKSRWQEGNVFSCSVMHEALHNHYTQKSLSLSLG

SEQ ID NO: 86 - protein, 447 aa, synthetic construct
EVQLVESGGGLVQPGGSLRLSCAASGFTFSGFGMNWVRQAPGKGLEWVSYTSSSSRTIYYADSVKGRFTISRDNAQNSLYLQMNSLRDEDTAVYYCARDSSGWYDAFDIWGQGTMVTVSSASTKGPSVFPLAPCSRSTSESTAALGCLVKDYFPEPVTVSWNSGALTSGVHTFPAVLQSSGLYSLSSVVTVPSSSLGTKTYTCNVDHKPSNTKVDKRVESKYGPPCPSCPAPEAAGGPSVFLFPPKPKDTLMISRTPEVTCVVVDVSQEDPEVQFNWYVDGVEVHNAKTKPREEQFNSTYRVVSVLTVLHQDWLNGKEYKCKVSNKGLPSSIEKTISKAKGQPREPQVYTLPPSQEEMTKNQVSLTCLVKGFYPSDIAVEWESNGQPENNYKTTPPVLDSDGSFFLYSRLTVDKSRWQEGNVFSCSVMHEALHNHYTQKSLSLSLGK

SEQ ID NO: 87 - protein, 446 aa, synthetic construct
EVQLVESGGGLVQPGGSLRLSCAASGFTFSGFGMNWVRQAPGKGLEWVSYTSSSSRTIYYADSVKGRFTISRDNAQNSLYLQMNSLRDEDTAVYYCARDSSGWYDAFDIWGQGTMVTVSSASTKGPSVFPLAPCSRSTSESTAALGCLVKDYFPEPVTVSWNSGALTSGVHTFPAVLQSSGLYSLSSVVTVPSSSLGTKTYTCNVDHKPSNTKVDKRVESKYGPPCPSCPAPEAAGGPSVFLFPPKPKDTLMISRTPEVTCVVVDVSQEDPEVQFNWYVDGVEVHNAKTKPREEQFNSTYRVVSVLTVLHQDWLNGKEYKCKVSNKGLPSSIEKTISKAKGQPREPQVYTLPPSQEEMTKNQVSLTCLVKGFYPSDIAVEWESNGQPENNYKTTPPVLDSDGSFFLYSRLTVDKSRWQEGNVFSCSVMHEALHNHYTQKSLSLSLG

SEQ ID NO: 88 - protein, 447 aa, synthetic construct
EVQLVESGGGLVQPGGSLRLSCAASGFTFSGFGMNWVRQAPGKGLEWVSYTSSSSRTIYYADSVKGRFTISRDNAQNSLYLQMNSLRDEDTAVYYCARDSSGWYDAFDIWGQGTMVTVSSASTKGPSVFPLAPCSRSTSESTAALGCLVKDYFPEPVTVSWNSGALTSGVHTFPAVLQSSGLYSLSSVVTVPSSSLGTKTYTCNVDHKPSNTKVDKRVESKYGPPCPSCPAPEFLGGPSVFLFPPKPKDTLYITREPEVTCVVVDVSQEDPEVQFNWYVDGVEVHNAKTKPREEQFNSTYRVVSVLTVLHQDWLNGKEYKCKVSNKGLPSSIEKTISKAKGQPREPQVYTLPPSQEEMTKNQVSLTCLVKGFYPSDIAVEWESNGQPENNYKTTPPVLDSDGSFFLYSRLTVDKSRWQEGNVFSCSVMHEALHNHYTQKSLSLSLGK

SEQ ID NO: 89 - protein, 446 aa, synthetic construct
EVQLVESGGGLVQPGGSLRLSCAASGFTFSGFGMNWVRQAPGKGLEWVSYTSSSSRTIYYADSVKGRFTISRDNAQNSLYLQMNSLRDEDTAVYYCARDSSGWYDAFDIWGQGTMVTVSSASTKGPSVFPLAPCSRSTSESTAALGCLVKDYFPEPVTVSWNSGALTSGVHTFPAVLQSSGLYSLSSVVTVPSSSLGTKTYTCNVDHKPSNTKVDKRVESKYGPPCPSCPAPEFLGGPSVFLFPPKPKDTLYITREPEVTCVVVDVSQEDPEVQFNWYVDGVEVHNAKTKPREEQFNSTYRVVSVLTVLHQDWLNGKEYKCKVSNKGLPSSIEKTISKAKGQPREPQVYTLPPSQEEMTKNQVSLTCLVKGFYPSDIAVEWESNGQPENNYKTTPPVLDSDGSFFLYSRLTVDKSRWQEGNVFSCSVMHEALHNHYTQKSLSLSLG

SEQ ID NO: 90 - protein, 447 aa, synthetic construct
EVQLVESGGGLVQPGGSLRLSCAASGFTFSGFGMNWVRQAPGKGLEWVSYTSSSSRTIYYADSVKGRFTISRDNAQNSLYLQMNSLRDEDTAVYYCARDSSGWYDAFDIWGQGTMVTVSSASTKGPSVFPLAPCSRSTSESTAALGCLVKDYFPEPVTVSWNSGALTSGVHTFPAVLQSSGLYSLSSVVTVPSSSLGTKTYTCNVDHKPSNTKVDKRVESKYGPPCPSCPAPESTRGPSVFLFPPKPKDTLYITREPEVTCVVVDVSQEDPEVQFNWYVDGVEVHNAKTKPREEQFNSTYRVVSVLTVLHQDWLNGKEYKCKVSNKGLPSSIEKTISKAKGQPREPQVYTLPPSQEEMTKNQVSLTCLVKGFYPSDIAVEWESNGQPENNYKTTPPVLDSDGSFFLYSRLTVDKSRWQEGNVFSCSVMHEALHNHYTQKSLSLSLGK

SEQ ID NO: 91 - protein, 446 aa, synthetic construct
EVQLVESGGGLVQPGGSLRLSCAASGFTFSGFGMNWVRQAPGKGLEWVSYTSSSSRTIYYADSVKGRFTISRDNAQNSLYLQMNSLRDEDTAVYYCARDSSGWYDAFDIWGQGTMVTVSSASTKGPSVFPLAPCSRSTSESTAALGCLVKDYFPEPVTVSWNSGALTSGVHTFPAVLQSSGLYSLSSVVTVPSSSLGTKTYTCNVDHKPSNTKVDKRVESKYGPPCPSCPAPESTRGPSVFLFPPKPKDTLYITREPEVTCVVVDVSQEDPEVQFNWYVDGVEVHNAKTKPREEQFNSTYRVVSVLTVLHQDWLNGKEYKCKVSNKGLPSSIEKTISKAKGQPREPQVYTLPPSQEEMTKNQVSLTCLVKGFYPSDIAVEWESNGQPENNYKTTPPVLDSDGSFFLYSRLTVDKSRWQEGNVFSCSVMHEALHNHYTQKSLSLSLG

SEQ ID NO: 92 - protein, 447 aa, synthetic construct
EVQLVESGGGLVQPGGSLRLSCAASGFTFSGFGMNWVRQAPGKGLEWVSYTSSSSRTIYYADSVKGRFTISRDNAQNSLYLQMNSLRDEDTAVYYCARDSSGWYDAFDIWGQGTMVTVSSASTKGPSVFPLAPCSRSTSESTAALGCLVKDYFPEPVTVSWNSGALTSGVHTFPAVLQSSGLYSLSSVVTVPSSSLGTKTYTCNVDHKPSNTKVDKRVESKYGPPCPSCPAPEAAGGPSVFLFPPKPKDTLYITREPEVTCVVVDVSQEDPEVQFNWYVDGVEVHNAKTKPREEQFNSTYRVVSVLTVLHQDWLNGKEYKCKVSNKGLPSSIEKTISKAKGQPREPQVYTLPPSQEEMTKNQVSLTCLVKGFYPSDIAVEWESNGQPENNYKTTPPVLDSDGSFFLYSRLTVDKSRWQEGNVFSCSVMHEALHNHYTQKSLSLSLGK

SEQ ID NO: 93 - protein, 446 aa, synthetic construct
EVQLVESGGGLVQPGGSLRLSCAASGFTFSGFGMNWVRQAPGKGLEWVSYTSSSSRTIYYADSVKGRFTISRDNAQNSLYLQMNSLRDEDTAVYYCARDSSGWYDAFDIWGQGTMVTVSSASTKGPSVFPLAPCSRSTSESTAALGCLVKDYFPEPVTVSWNSGALTSGVHTFPAVLQSSGLYSLSSVVTVPSSSLGTKTYTCNVDHKPSNTKVDKRVESKYGPPCPSCPAPEAAGGPSVFLFPPKPKDTLYITREPEVTCVVVDVSQEDPEVQFNWYVDGVEVHNAKTKPREEQFNSTYRVVSVLTVLHQDWLNGKEYKCKVSNKGLPSSIEKTISKAKGQPREPQVYTLPPSQEEMTKNQVSLTCLVKGFYPSDIAVEWESNGQPENNYKTTPPVLDSDGSFFLYSRLTVDKSRWQEGNVFSCSVMHEALHNHYTQKSLSLSLG

SEQ ID NO: 94 - protein, 447 aa, synthetic construct
EVQLVESGGGLVQPGGSLRLSCAASGFTFSGFGMNWVRQAPGKGLEWVSYTSSSSRTIYYADSVKGRFTISRDNAQNSLYLQMNSLRDEDTAVYYCARDSSGWYDAFDIWGQGTMVTVSSASTKGPSVFPLAPCSRSTSESTAALGCLVKDYFPEPVTVSWNSGALTSGVHTFPAVLQSSGLYSLSSVVTVPSSSLGTKTYTCNVDHKPSNTKVDKRVESKYGPPCPSCPAPEFLGGPSVFLFPPKPKDTLMISRTPEVTCVVVDVSQEDPEVQFNWYVDGVEVHNAKTKPREEQFNSTYRVVSVLTVLHRDWLNGKEYKCKVSNKGLPSSIEKTISKAKGQPREPQVYTLPPSQEEMTKNQVSLTCLVKGFYPSDIAVEWESNGQPENNYKTTPPVLDSDGSFFLYSRLTVDKSRWQEGNVFSCSVEHEALHWHYTQKSLSLSLGK

SEQ ID NO: 95 - protein, 446 aa, synthetic construct
EVQLVESGGGLVQPGGSLRLSCAASGFTFSGFGMNWVRQAPGKGLEWVSYTSSSSRTIYYADSVKGRFTISRDNAQNSLYLQMNSLRDEDTAVYYCARDSSGWYDAFDIWGQGTMVTVSSASTKGPSVFPLAPCSRSTSESTAALGCLVKDYFPEPVTVSWNSGALTSGVHTFPAVLQSSGLYSLSSVVTVPSSSLGTKTYTCNVDHKPSNTKVDKRVESKYGPPCPSCPAPEFLGGPSVFLFPPKPKDTLMISRTPEVTCVVVDVSQEDPEVQFNWYVDGVEVHNAKTKPREEQFNSTYRVVSVLTVLHRDWLNGKEYKCKVSNKGLPSSIEKTISKAKGQPREPQVYTLPPSQEEMTKNQVSLTCLVKGFYPSDIAVEWESNGQPENNYKTTPPVLDSDGSFFLYSRLTVDKSRWQEGNVFSCSVEHEALHWHYTQKSLSLSLG

SEQ ID NO: 96 - protein, 447 aa, synthetic construct
EVQLVESGGGLVQPGGSLRLSCAASGFTFSGFGMNWVRQAPGKGLEWVSYTSSSSRTIYYADSVKGRFTISRDNAQNSLYLQMNSLRDEDTAVYYCARDSSGWYDAFDIWGQGTMVTVSSASTKGPSVFPLAPCSRSTSESTAALGCLVKDYFPEPVTVSWNSGALTSGVHTFPAVLQSSGLYSLSSVVTVPSSSLGTKTYTCNVDHKPSNTKVDKRVESKYGPPCPSCPAPESTRGPSVFLFPPKPKDTLMISRTPEVTCVVVDVSQEDPEVQFNWYVDGVEVHNAKTKPREEQFNSTYRVVSVLTVLHRDWLNGKEYKCKVSNKGLPSSIEKTISKAKGQPREPQVYTLPPSQEEMTKNQVSLTCLVKGFYPSDIAVEWESNGQPENNYKTTPPVLDSDGSFFLYSRLTVDKSRWQEGNVFSCSVEHEALHWHYTQKSLSLSLGK

SEQ ID NO: 97 - protein, 446 aa, synthetic construct
EVQLVESGGGLVQPGGSLRLSCAASGFTFSGFGMNWVRQAPGKGLEWVSYTSSSSRTIYYADSVKGRFTISRDNAQNSLYLQMNSLRDEDTAVYYCARDSSGWYDAFDIWGQGTMVTVSSASTKGPSVFPLAPCSRSTSESTAALGCLVKDYFPEPVTVSWNSGALTSGVHTFPAVLQSSGLYSLSSVVTVPSSSLGTKTYTCNVDHKPSNTKVDKRVESKYGPPCPSCPAPESTRGPSVFLFPPKPKDTLMISRTPEVTCVVVDVSQEDPEVQFNWYVDGVEVHNAKTKPREEQFNSTYRVVSVLTVLHRDWLNGKEYKCKVSNKGLPSSIEKTISKAKGQPREPQVYTLPPSQEEMTKNQVSLTCLVKGFYPSDIAVEWESNGQPENNYKTTPPVLDSDGSFFLYSRLTVDKSRWQEGNVFSCSVEHEALHWHYTQKSLSLSLG

SEQ ID NO: 98 - protein, 447 aa, synthetic construct
EVQLVESGGGLVQPGGSLRLSCAASGFTFSGFGMNWVRQAPGKGLEWVSYTSSSSRTIYYADSVKGRFTISRDNAQNSLYLQMNSLRDEDTAVYYCARDSSGWYDAFDIWGQGTMVTVSSASTKGPSVFPLAPCSRSTSESTAALGCLVKDYFPEPVTVSWNSGALTSGVHTFPAVLQSSGLYSLSSVVTVPSSSLGTKTYTCNVDHKPSNTKVDKRVESKYGPPCPSCPAPEAAGGPSVFLFPPKPKDTLMISRTPEVTCVVVDVSQEDPEVQFNWYVDGVEVHNAKTKPREEQFNSTYRVVSVLTVLHRDWLNGKEYKCKVSNKGLPSSIEKTISKAKGQPREPQVYTLPPSQEEMTKNQVSLTCLVKGFYPSDIAVEWESNGQPENNYKTTPPVLDSDGSFFLYSRLTVDKSRWQEGNVFSCSVEHEALHWHYTQKSLSLSLGK

SEQ ID NO: 99 - protein, 446 aa, synthetic construct
EVQLVESGGGLVQPGGSLRLSCAASGFTFSGFGMNWVRQAPGKGLEWVSYTSSSSRTIYYADSVKGRFTISRDNAQNSLYLQMNSLRDEDTAVYYCARDSSGWYDAFDIWGQGTMVTVSSASTKGPSVFPLAPCSRSTSESTAALGCLVKDYFPEPVTVSWNSGALTSGVHTFPAVLQSSGLYSLSSVVTVPSSSLGTKTYTCNVDHKPSNTKVDKRVESKYGPPCPSCPAPEAAGGPSVFLFPPKPKDTLMISRTPEVTCVVVDVSQEDPEVQFNWYVDGVEVHNAKTKPREEQFNSTYRVVSVLTVLHRDWLNGKEYKCKVSNKGLPSSIEKTISKAKGQPREPQVYTLPPSQEEMTKNQVSLTCLVKGFYPSDIAVEWESNGQPENNYKTTPPVLDSDGSFFLYSRLTVDKSRWQEGNVFSCSVEHEALHWHYTQKSLSLSLG

SEQ ID NO: 100 - protein, 447 aa, synthetic construct
EVQLVESGGGLVQPGGSLRLSCAASGFTFSGFGMNWVRQAPGKGLEWVSYTSSSSRTIYYADSVKGRFTISRDNAQNSLYLQMNSLRDEDTAVYYCARDSSGWYDAFDIWGQGTMVTVSSASTKGPSVFPLAPCSRSTSESTAALGCLVKDYFPEPVTVSWNSGALTSGVHTFPAVLQSSGLYSLSSVVTVPSSSLGTKTYTCNVDHKPSNTKVDKRVESKYGPPCPSCPAPEFLGGPSVFLFPPKPKDTLMISRTPEVTCVVVDVSQEDPEVQFNWYVDGVEVHNAKTKPREEQFNSTYRVVSVLTVLHQDWLNGKEYKCKVSNKGLPSSIEKTISKAKGQPREPQVYTLPPSQEEMTKNQVSLTCLVKGFYPSDIAVEWESNGQPENNYKTTPPVLDSDGSFFLYSRLTVDKSRWQEGNVFSCSVLHEALHSHYTQKSLSLSLGK

SEQ ID NO: 101 - protein, 446 aa, synthetic construct
EVQLVESGGGLVQPGGSLRLSCAASGFTFSGFGMNWVRQAPGKGLEWVSYTSSSSRTIYYADSVKGRFTISRDNAQNSLYLQMNSLRDEDTAVYYCARDSSGWYDAFDIWGQGTMVTVSSASTKGPSVFPLAPCSRSTSESTAALGCLVKDYFPEPVTVSWNSGALTSGVHTFPAVLQSSGLYSLSSVVTVPSSSLGTKTYTCNVDHKPSNTKVDKRVESKYGPPCPSCPAPEFLGGPSVFLFPPKPKDTLMISRTPEVTCVVVDVSQEDPEVQFNWYVDGVEVHNAKTKPREEQFNSTYRVVSVLTVLHQDWLNGKEYKCKVSNKGLPSSIEKTISKAKGQPREPQVYTLPPSQEEMTKNQVSLTCLVKGFYPSDIAVEWESNGQPENNYKTTPPVLDSDGSFFLYSRLTVDKSRWQEGNVFSCSVLHEALHSHYTQKSLSLSLG

SEQ ID NO: 102 - protein, 447 aa, synthetic construct
EVQLVESGGGLVQPGGSLRLSCAASGFTFSGFGMNWVRQAPGKGLEWVSYTSSSSRTIYYADSVKGRFTISRDNAQNSLYLQMNSLRDEDTAVYYCARDSSGWYDAFDIWGQGTMVTVSSASTKGPSVFPLAPCSRSTSESTAALGCLVKDYFPEPVTVSWNSGALTSGVHTFPAVLQSSGLYSLSSVVTVPSSSLGTKTYTCNVDHKPSNTKVDKRVESKYGPPCPSCPAPESTRGPSVFLFPPKPKDTLMISRTPEVTCVVVDVSQEDPEVQFNWYVDGVEVHNAKTKPREEQFNSTYRVVSVLTVLHQDWLNGKEYKCKVSNKGLPSSIEKTISKAKGQPREPQVYTLPPSQEEMTKNQVSLTCLVKGFYPSDIAVEWESNGQPENNYKTTPPVLDSDGSFFLYSRLTVDKSRWQEGNVFSCSVLHEALHSHYTQKSLSLSLGK

SEQ ID NO: 103 - protein, 446 aa, synthetic construct
EVQLVESGGGLVQPGGSLRLSCAASGFTFSGFGMNWVRQAPGKGLEWVSYTSSSSRTIYYADSVKGRFTISRDNAQNSLYLQMNSLRDEDTAVYYCARDSSGWYDAFDIWGQGTMVTVSSASTKGPSVFPLAPCSRSTSESTAALGCLVKDYFPEPVTVSWNSGALTSGVHTFPAVLQSSGLYSLSSVVTVPSSSLGTKTYTCNVDHKPSNTKVDKRVESKYGPPCPSCPAPESTRGPSVFLFPPKPKDTLMISRTPEVTCVVVDVSQEDPEVQFNWYVDGVEVHNAKTKPREEQFNSTYRVVSVLTVLHQDWLNGKEYKCKVSNKGLPSSIEKTISKAKGQPREPQVYTLPPSQEEMTKNQVSLTCLVKGFYPSDIAVEWESNGQPENNYKTTPPVLDSDGSFFLYSRLTVDKSRWQEGNVFSCSVLHEALHSHYTQKSLSLSLG

SEQ ID NO: 104 - protein, 447 aa, synthetic construct
EVQLVESGGGLVQPGGSLRLSCAASGFTFSGFGMNWVRQAPGKGLEWVSYTSSSSRTIYYADSVKGRFTISRDNAQNSLYLQMNSLRDEDTAVYYCARDSSGWYDAFDIWGQGTMVTVSSASTKGPSVFPLAPCSRSTSESTAALGCLVKDYFPEPVTVSWNSGALTSGVHTFPAVLQSSGLYSLSSVVTVPSSSLGTKTYTCNVDHKPSNTKVDKRVESKYGPPCPSCPAPEAAGGPSVFLFPPKPKDTLMISRTPEVTCVVVDVSQEDPEVQFNWYVDGVEVHNAKTKPREEQFNSTYRVVSVLTVLHQDWLNGKEYKCKVSNKGLPSSIEKTISKAKGQPREPQVYTLPPSQEEMTKNQVSLTCLVKGFYPSDIAVEWESNGQPENNYKTTPPVLDSDGSFFLYSRLTVDKSRWQEGNVFSCSVLHEALHSHYTQKSLSLSLGK

SEQ ID NO: 105 - protein, 446 aa, synthetic construct
EVQLVESGGGLVQPGGSLRLSCAASGFTFSGFGMNWVRQAPGKGLEWVSYTSSSSRTIYYADSVKGRFTISRDNAQNSLYLQMNSLRDEDTAVYYCARDSSGWYDAFDIWGQGTMVTVSSASTKGPSVFPLAPCSRSTSESTAALGCLVKDYFPEPVTVSWNSGALTSGVHTFPAVLQSSGLYSLSSVVTVPSSSLGTKTYTCNVDHKPSNTKVDKRVESKYGPPCPSCPAPEAAGGPSVFLFPPKPKDTLMISRTPEVTCVVVDVSQEDPEVQFNWYVDGVEVHNAKTKPREEQFNSTYRVVSVLTVLHQDWLNGKEYKCKVSNKGLPSSIEKTISKAKGQPREPQVYTLPPSQEEMTKNQVSLTCLVKGFYPSDIAVEWESNGQPENNYKTTPPVLDSDGSFFLYSRLTVDKSRWQEGNVFSCSVLHEALHSHYTQKSLSLSLG

SEQ ID NO: 106 - protein, 447 aa, synthetic construct
EVQLVESGGGLVQPGGSLRLSCAASGFTFSGFGMNWVRQAPGKGLEWVSYTSSSSRTIYYADSVKGRFTISRDNAQNSLYLQMNSLRDEDTAVYYCARDSSGWYDAFDIWGQGTMVTVSSASTKGPSVFPLAPCSRSTSESTAALGCLVKDYFPEPVTVSWNSGALTSGVHTFPAVLQSSGLYSLSSVVTVPSSSLGTKTYTCNVDHKPSNTKVDKRVESKYGPPCPSCPAPEFLGGPSVFLFPPKPKDQLMISRTPEVTCVVVDVSQEDPEVQFNWYVDGVEVHNAKTKPREEQFNSTYRVVSVLTVLHQDWLNGKEYKCKVSNKGLPSSIEKTISKAKGQPREPQVYTLPPSQEEMTKNQVSLTCLVKGFYPSDIAVEWESNGQPENNYKTTPPVLDSDGSFFLYSRLTVDKSRWQEGNVFSCSVLHEALHNHYTQKSLSLSLGK

SEQ ID NO: 107 - protein, 446 aa, synthetic construct
EVQLVESGGGLVQPGGSLRLSCAASGFTFSGFGMNWVRQAPGKGLEWVSYTSSSSRTIYYADSVKGRFTISRDNAQNSLYLQMNSLRDEDTAVYYCARDSSGWYDAFDIWGQGTMVTVSSASTKGPSVFPLAPCSRSTSESTAALGCLVKDYFPEPVTVSWNSGALTSGVHTFPAVLQSSGLYSLSSVVTVPSSSLGTKTYTCNVDHKPSNTKVDKRVESKYGPPCPSCPAPEFLGGPSVFLFPPKPKDQLMISRTPEVTCVVVDVSQEDPEVQFNWYVDGVEVHNAKTKPREEQFNSTYRVVSVLTVLHQDWLNGKEYKCKVSNKGLPSSIEKTISKAKGQPREPQVYTLPPSQEEMTKNQVSLTCLVKGFYPSDIAVEWESNGQPENNYKTTPPVLDSDGSFFLYSRLTVDKSRWQEGNVFSCSVLHEALHNHYTQKSLSLSLG

SEQ ID NO: 108 - protein, 447 aa, synthetic construct
EVQLVESGGGLVQPGGSLRLSCAASGFTFSGFGMNWVRQAPGKGLEWVSYTSSSSRTIYYADSVKGRFTISRDNAQNSLYLQMNSLRDEDTAVYYCARDSSGWYDAFDIWGQGTMVTVSSASTKGPSVFPLAPCSRSTSESTAALGCLVKDYFPEPVTVSWNSGALTSGVHTFPAVLQSSGLYSLSSVVTVPSSSLGTKTYTCNVDHKPSNTKVDKRVESKYGPPCPSCPAPESTRGPSVFLFPPKPKDQLMISRTPEVTCVVVDVSQEDPEVQFNWYVDGVEVHNAKTKPREEQFNSTYRVVSVLTVLHQDWLNGKEYKCKVSNKGLPSSIEKTISKAKGQPREPQVYTLPPSQEEMTKNQVSLTCLVKGFYPSDIAVEWESNGQPENNYKTTPPVLDSDGSFFLYSRLTVDKSRWQEGNVFSCSVLHEALHNHYTQKSLSLSLGK

SEQ ID NO: 109 - protein, 446 aa, synthetic construct
EVQLVESGGGLVQPGGSLRLSCAASGFTFSGFGMNWVRQAPGKGLEWVSYTSSSSRTIYYADSVKGRFTISRDNAQNSLYLQMNSLRDEDTAVYYCARDSSGWYDAFDIWGQGTMVTVSSASTKGPSVFPLAPCSRSTSESTAALGCLVKDYFPEPVTVSWNSGALTSGVHTFPAVLQSSGLYSLSSVVTVPSSSLGTKTYTCNVDHKPSNTKVDKRVESKYGPPCPSCPAPESTRGPSVFLFPPKPKDQLMISRTPEVTCVVVDVSQEDPEVQFNWYVDGVEVHNAKTKPREEQFNSTYRVVSVLTVLHQDWLNGKEYKCKVSNKGLPSSIEKTISKAKGQPREPQVYTLPPSQEEMTKNQVSLTCLVKGFYPSDIAVEWESNGQPENNYKTTPPVLDSDGSFFLYSRLTVDKSRWQEGNVFSCSVLHEALHNHYTQKSLSLSLG

SEQ ID NO: 110 - protein, 447 aa, synthetic construct
EVQLVESGGGLVQPGGSLRLSCAASGFTFSGFGMNWVRQAPGKGLEWVSYTSSSSRTIYYADSVKGRFTISRDNAQNSLYLQMNSLRDEDTAVYYCARDSSGWYDAFDIWGQGTMVTVSSASTKGPSVFPLAPCSRSTSESTAALGCLVKDYFPEPVTVSWNSGALTSGVHTFPAVLQSSGLYSLSSVVTVPSSSLGTKTYTCNVDHKPSNTKVDKRVESKYGPPCPSCPAPEAAGGPSVFLFPPKPKDQLMISRTPEVTCVVVDVSQEDPEVQFNWYVDGVEVHNAKTKPREEQFNSTYRVVSVLTVLHQDWLNGKEYKCKVSNKGLPSSIEKTISKAKGQPREPQVYTLPPSQEEMTKNQVSLTCLVKGFYPSDIAVEWESNGQPENNYKTTPPVLDSDGSFFLYSRLTVDKSRWQEGNVFSCSVLHEALHNHYTQKSLSLSLGK

SEQ ID NO: 111 - protein, 446 aa, synthetic construct
EVQLVESGGGLVQPGGSLRLSCAASGFTFSGFGMNWVRQAPGKGLEWVSYTSSSSRTIYYADSVKGRFTISRDNAQNSLYLQMNSLRDEDTAVYYCARDSSGWYDAFDIWGQGTMVTVSSASTKGPSVFPLAPCSRSTSESTAALGCLVKDYFPEPVTVSWNSGALTSGVHTFPAVLQSSGLYSLSSVVTVPSSSLGTKTYTCNVDHKPSNTKVDKRVESKYGPPCPSCPAPEAAGGPSVFLFPPKPKDQLMISRTPEVTCVVVDVSQEDPEVQFNWYVDGVEVHNAKTKPREEQFNSTYRVVSVLTVLHQDWLNGKEYKCKVSNKGLPSSIEKTISKAKGQPREPQVYTLPPSQEEMTKNQVSLTCLVKGFYPSDIAVEWESNGQPENNYKTTPPVLDSDGSFFLYSRLTVDKSRWQEGNVFSCSVLHEALHNHYTQKSLSLSLG

SEQ ID NO: 112 - protein, 447 aa, synthetic construct
EVQLVESGGGLVQPGGSLRLSCAASGFTFSGFGMNWVRQAPGKGLEWVSYTSSSSRTIYYADSVKGRFTISRDNAQNSLYLQMNSLRDEDTAVYYCARDSSGWYDAFDIWGQGTMVTVSSASTKGPSVFPLAPCSRSTSESTAALGCLVKDYFPEPVTVSWNSGALTSGVHTFPAVLQSSGLYSLSSVVTVPSSSLGTKTYTCNVDHKPSNTKVDKRVESKYGPPCPSCPAPEFLGGPSVFLFPPKPKDTLMISRTPEVTCVVVDVSQEDPEVQFNWYVDGVEVHNAKTKPREEQFNSTYRVVSVLTVDHHDWLNGKEYKCKVSNKGLPSSIEKTISKAKGQPREPQVYTLPPSQEEMTKNQVSLTCLVKGFYPSDIAVEWESNGQPENNYKTTPPVLDSDGSFFLYSRLTVDKSRWQEGNVFSCSVMHEALHSHYTQKSLSLSLGK

SEQ ID NO: 113 - protein, 446 aa, synthetic construct
EVQLVESGGGLVQPGGSLRLSCAASGFTFSGFGMNWVRQAPGKGLEWVSYTSSSSRTIYYADSVKGRFTISRDNAQNSLYLQMNSLRDEDTAVYYCARDSSGWYDAFDIWGQGTMVTVSSASTKGPSVFPLAPCSRSTSESTAALGCLVKDYFPEPVTVSWNSGALTSGVHTFPAVLQSSGLYSLSSVVTVPSSSLGTKTYTCNVDHKPSNTKVDKRVESKYGPPCPSCPAPEFLGGPSVFLFPPKPKDTLMISRTPEVTCVVVDVSQEDPEVQFNWYVDGVEVHNAKTKPREEQFNSTYRVVSVLTVDHHDWLNGKEYKCKVSNKGLPSSIEKTISKAKGQPREPQVYTLPPSQEEMTKNQVSLTCLVKGFYPSDIAVEWESNGQPENNYKTTPPVLDSDGSFFLYSRLTVDKSRWQEGNVFSCSVMHEALHSHYTQKSLSLSLG

SEQ ID NO: 114 - protein, 447 aa, synthetic construct
EVQLVESGGGLVQPGGSLRLSCAASGFTFSGFGMNWVRQAPGKGLEWVSYTSSSSRTIYYADSVKGRFTISRDNAQNSLYLQMNSLRDEDTAVYYCARDSSGWYDAFDIWGQGTMVTVSSASTKGPSVFPLAPCSRSTSESTAALGCLVKDYFPEPVTVSWNSGALTSGVHTFPAVLQSSGLYSLSSVVTVPSSSLGTKTYTCNVDHKPSNTKVDKRVESKYGPPCPSCPAPESTRGPSVFLFPPKPKDTLMISRTPEVTCVVVDVSQEDPEVQFNWYVDGVEVHNAKTKPREEQFNSTYRVVSVLTVDHHDWLNGKEYKCKVSNKGLPSSIEKTISKAKGQPREPQVYTLPPSQEEMTKNQVSLTCLVKGFYPSDIAVEWESNGQPENNYKTTPPVLDSDGSFFLYSRLTVDKSRWQEGNVFSCSVMHEALHSHYTQKSLSLSLGK

SEQ ID NO: 115 - protein, 446 aa, synthetic construct
EVQLVESGGGLVQPGGSLRLSCAASGFTFSGFGMNWVRQAPGKGLEWVSYTSSSSRTIYYADSVKGRFTISRDNAQNSLYLQMNSLRDEDTAVYYCARDSSGWYDAFDIWGQGTMVTVSSASTKGPSVFPLAPCSRSTSESTAALGCLVKDYFPEPVTVSWNSGALTSGVHTFPAVLQSSGLYSLSSVVTVPSSSLGTKTYTCNVDHKPSNTKVDKRVESKYGPPCPSCPAPESTRGPSVFLFPPKPKDTLMISRTPEVTCVVVDVSQEDPEVQFNWYVDGVEVHNAKTKPREEQFNSTYRVVSVLTVDHHDWLNGKEYKCKVSNKGLPSSIEKTISKAKGQPREPQVYTLPPSQEEMTKNQVSLTCLVKGFYPSDIAVEWESNGQPENNYKTTPPVLDSDGSFFLYSRLTVDKSRWQEGNVFSCSVMHEALHSHYTQKSLSLSLG

SEQ ID NO: 116 - protein, 447 aa, synthetic construct
EVQLVESGGGLVQPGGSLRLSCAASGFTFSGFGMNWVRQAPGKGLEWVSYTSSSSRTIYYADSVKGRFTISRDNAQNSLYLQMNSLRDEDTAVYYCARDSSGWYDAFDIWGQGTMVTVSSASTKGPSVFPLAPCSRSTSESTAALGCLVKDYFPEPVTVSWNSGALTSGVHTFPAVLQSSGLYSLSSVVTVPSSSLGTKTYTCNVDHKPSNTKVDKRVESKYGPPCPSCPAPEAAGGPSVFLFPPKPKDTLMISRTPEVTCVVVDVSQEDPEVQFNWYVDGVEVHNAKTKPREEQFNSTYRVVSVLTVDHHDWLNGKEYKCKVSNKGLPSSIEKTISKAKGQPREPQVYTLPPSQEEMTKNQVSLTCLVKGFYPSDIAVEWESNGQPENNYKTTPPVLDSDGSFFLYSRLTVDKSRWQEGNVFSCSVMHEALHSHYTQKSLSLSLGK

SEQ ID NO: 117 - protein, 446 aa, synthetic construct
EVQLVESGGGLVQPGGSLRLSCAASGFTFSGFGMNWVRQAPGKGLEWVSYTSSSSRTIYYADSVKGRFTISRDNAQNSLYLQMNSLRDEDTAVYYCARDSSGWYDAFDIWGQGTMVTVSSASTKGPSVFPLAPCSRSTSESTAALGCLVKDYFPEPVTVSWNSGALTSGVHTFPAVLQSSGLYSLSSVVTVPSSSLGTKTYTCNVDHKPSNTKVDKRVESKYGPPCPSCPAPEAAGGPSVFLFPPKPKDTLMISRTPEVTCVVVDVSQEDPEVQFNWYVDGVEVHNAKTKPREEQFNSTYRVVSVLTVDHHDWLNGKEYKCKVSNKGLPSSIEKTISKAKGQPREPQVYTLPPSQEEMTKNQVSLTCLVKGFYPSDIAVEWESNGQPENNYKTTPPVLDSDGSFFLYSRLTVDKSRWQEGNVFSCSVMHEALHSHYTQKSLSLSLG